European Patent Application EP 4 176 895 A1, published May 10, 2023. Title: Targeting modules against IL13RA2 and/or HER2 for use in a method for stimulating a chimeric antigen receptor-mediated immune response in a mammal. Applicant: GEMoaB GmbH. The sequence listing filed with the application follows.

SEQUENCE LISTING (176 sequences)

SEQ ID NO: 1 - protein, 112 aa, Homo sapiens
GPVPPSTALRELIEELVNITQNQKAPLCNGSMVWSINLTAGMYCAALESLINVSGCSAIEKTQRMLSGFCPHKVSAGQFSSLHVRDTKIEVAQFVKDLLLHLKKLFREGRFN

SEQ ID NO: 2 - protein, 112 aa, Homo sapiens
GPVPPSTALRYLIEELVNITQNQKAPLCNYSMVWSINLTAGMYCAALESLINVSGCSAIEKTQRMLSGFCPHKVSAGQFSSLHVRDTKIEVAQFVKDLLLHLKKLFREGRFN

SEQ ID NO: 3 - protein, 112 aa, Homo sapiens
GPVPPSTALRYLIEELVNITQNQKAPLCNGSAVWSINLTAGMYCAALESLINVSGCSAIEKTQRMLSGFCPHKVSAGQFSSLHVRDTKIEVAQFVKDLLLHLKKLFREGRFN

SEQ ID NO: 4 - protein, 112 aa, Homo sapiens
  Xaa can be any naturally occurring amino acid (1)..(32)
GPVPPSTALRXLIEELVNITQNQKAPLCNXSXVWSINLTAGMYCAALESLINVSGCSAIEKTQRMLSGFCPHKVSAGQFSSLHVRDTKIEVAQFVKDLLLHLKKLFREGRFN

SEQ ID NO: 5 - protein, 242 aa, Mus musculus
EFQVQLQQPGAELVKPGASVKLSCKASGYTFTSHWIHWVKERPGRGLEWIGRIEPNSGGTLYNEKFKTKATLTVDKPSSTAYMQINSLTSEDFAVYYCARWREFDFFDYWGQGTTLTVSSGGGGSGGGGSGGGGSDIVLTQSPATLSVTPGDSVSLSCRASQSISNNLHWYQQKSHESPRLLIKYASQSISGIPSRFSGSGSGTDFTLSISSVETEDFGMYFCQQSNRWPYTFGGGTKLEIK

SEQ ID NO: 6 - protein, 250 aa, Artificial Sequence
  humanized scFv
DIVLTQSPAFLSVTPGEKVTLTCQASQSISNNLHWYQQKPDQAPKLLIKYASQSISGVPSRFSGSGSGTDFTLTISSVEAEDFGTYYCQQSNRWPYTFGGGTKLEIKGGGGSGGGGSGASAAGGGGSGGGGSQVQLVQSGAEVVKPGASVKLSCKASGYTFTSHWIHWVKQAPGQGLEWIGRIEPNSGGTLYAQKFQGRATLTVDTSISTAYMEISRLRSDDTAVYYCARWREFDFFDYWGQGTTLTVSS

SEQ ID NO: 7 - protein, 250 aa, Artificial Sequence
  humanized scFv
DIVLTQSPAFLSVTPGEKVTLTCRASQSISNNLHWYQQKPDQAPKLLIKYASQSISGVPSRFSGSGSGTDFTLTISSVEAEDFGTYYCQQSNRWPYTFGGGTKLEIKGGGGSGGGGSGASAAGGGGSGGGGSQVQLVQSGAEVVKPGASVKLSCKASGYTFTSHWIHWVKQAPGQGLEWIGRIEPNSGGTLYNQKFQGRATLTVDKPSSTAYMEISRLRSDDTAVYYCARWREFDFFDYWGQGTTLTVSS

SEQ ID NO: 8 - protein, 250 aa, Artificial Sequence
  humanized scFv
DIVLTQSPAFLSVTPGEKVTLTCRASQSISNNLHWYQQKPDQAPKLLIKYASQSISGVPSRFSGSGSGTDFTLTISSVEAEDFGTYYCQQSNRWPYTFGGGTKLEIKGGGGSGGGGSGASAAGGGGSGGGGSQVQLVQSGAEVVKPGASVKLSCKASGYTFTSHWIHWVKQAPGQGLEWIGRIEPNSGGTLYNEKFKTRATLTVDKSISTAYMEISRLRSDDTAVYYCARWREFDFFDYWGQGTTLTVSS

SEQ ID NO: 9 - protein, 250 aa, Artificial Sequence
  humanized scFv
DVVMTQSPAFLSVTPGEKVTITCQASQSISNNLHWYQQKPDQAPKLLIKYASQSISGVPSRFSGSGSGTDFTFTISSLEAEDAATYFCQQSNRWPYTFGGGTKLEIKGGGGSGGGGSGASAAGGGGSGGGGSQVQLVQSGAEVKKPGASVKVSCKASGYTFTSHWIHWVRQAPGQGLEWMGRIEPNSGGTLYAQKFQGRVTMTRDTSISTAYMELSRLRSDDTAVYYCARWREFDFFDYWGQGTTLTVSS

SEQ ID NO: 10 - protein, 250 aa, Artificial Sequence
  humanized scFv
QIVLTQSPATLSLSPGERATLSCRASQSISNNLHWYQQKPGQAPRLLIKYASQSISGVPDRFSGSGSGTDFTLTISRLEPEDFAVYYCQQSNRWPYTFGGGTKLEIKGGGGSGGGGSGASAAGGGGSGGGGSQVQLVQSGAEVKKPGASVKVSCKASGYTFTSHWIHWVRQAPGQGLEWIGRIEPNSGGTLYNEKFKGRVTMTRDTSTSTVYMELSSLRSEDTAVYYCARWREFDFFDYWGAGTTVTVSS

SEQ ID NO: 11 - protein, 8 aa, Mus musculus
GYTFTSHW

SEQ ID NO: 12 - protein, 8 aa, Mus musculus
IEPNSGGT

SEQ ID NO: 13 - protein, 11 aa, Mus musculus
ARWREFDFFDY

SEQ ID NO: 14 - protein, 6 aa, Mus musculus
QSISNN

SEQ ID NO: 15 - protein, 3 aa, Mus musculus
YAS

SEQ ID NO: 16 - protein, 9 aa, Mus musculus
QQSNRWPYT

SEQ ID NO: 17 - protein, 107 aa, Artificial Sequence
  humanized VL chain
  Xaa can be any naturally occurring amino acid (1)..(87)
XXVXTQSPAXLSXXPGEXXTXXCXASQSISNNLHWYQQKPXQAPKLLIKYASQSISGVPXRFSGSGSGTDFTXTISXXEXEDXXXYXCQQSNRWPYTFGGGTKLEIK

SEQ ID NO: 18 - protein, 118 aa, Artificial Sequence
  humanized VH chain
  Xaa can be any naturally occurring amino acid (12)..(114)
QVQLVQSGAEVXKPGASVKXSCKASGYTFTSHWIHWVXQAPGQGLEWXGRIEPNSGGTLYXXKFXXRXTXTXDXXXSTXYMEXSXLRSXDTAVYYCARWREFDFFDYWGXGTTXTVSS

SEQ ID NO: 19 - protein, 107 aa, Mus musculus
DIVLTQSPATLSVTPGDSVSLSCRASQSISNNLHWYQQKSHESPRLLIKYASQSISGIPSRFSGSGSGTDFTLSISSVETEDFGMYFCQQSNRWPYTFGGGTKLEIK

SEQ ID NO: 20 - protein, 107 aa, Artificial Sequence
  humanized VL chain
DIVLTQSPAFLSVTPGEKVTLTCQASQSISNNLHWYQQKPDQAPKLLIKYASQSISGVPSRFSGSGSGTDFTLTISSVEAEDFGTYYCQQSNRWPYTFGGGTKLEIK

SEQ ID NO: 21 - protein, 107 aa, Artificial Sequence
  humanized VL chain
DIVLTQSPAFLSVTPGEKVTLTCRASQSISNNLHWYQQKPDQAPKLLIKYASQSISGVPSRFSGSGSGTDFTLTISSVEAEDFGTYYCQQSNRWPYTFGGGTKLEIK

SEQ ID NO: 22 - protein, 107 aa, Artificial Sequence; identical to SEQ ID NO: 21
  humanized VL chain

SEQ ID NO: 23 - protein, 107 aa, Artificial Sequence
  humanized VL chain
DVVMTQSPAFLSVTPGEKVTITCQASQSISNNLHWYQQKPDQAPKLLIKYASQSISGVPSRFSGSGSGTDFTFTISSLEAEDAATYFCQQSNRWPYTFGGGTKLEIK

SEQ ID NO: 24 - protein, 107 aa, Artificial Sequence
  humanized VL chain
QIVLTQSPATLSLSPGERATLSCRASQSISNNLHWYQQKPGQAPRLLIKYASQSISGVPDRFSGSGSGTDFTLTISRLEPEDFAVYYCQQSNRWPYTFGGGTKLEIK

SEQ ID NO: 25 - protein, 120 aa, Mus musculus
EFQVQLQQPGAELVKPGASVKLSCKASGYTFTSHWIHWVKERPGRGLEWIGRIEPNSGGTLYNEKFKTKATLTVDKPSSTAYMQINSLTSEDFAVYYCARWREFDFFDYWGQGTTLTVSS

SEQ ID NO: 26 - protein, 118 aa, Artificial Sequence
  humanized VH chain
QVQLVQSGAEVVKPGASVKLSCKASGYTFTSHWIHWVKQAPGQGLEWIGRIEPNSGGTLYAQKFQGRATLTVDTSISTAYMEISRLRSDDTAVYYCARWREFDFFDYWGQGTTLTVSS

SEQ ID NO: 27 - protein, 118 aa, Artificial Sequence
  humanized VH chain
QVQLVQSGAEVVKPGASVKLSCKASGYTFTSHWIHWVKQAPGQGLEWIGRIEPNSGGTLYNQKFQGRATLTVDKPSSTAYMEISRLRSDDTAVYYCARWREFDFFDYWGQGTTLTVSS

SEQ ID NO: 28 - protein, 118 aa, Artificial Sequence
  humanized VH chain
QVQLVQSGAEVVKPGASVKLSCKASGYTFTSHWIHWVKQAPGQGLEWIGRIEPNSGGTLYNEKFKTRATLTVDKSISTAYMEISRLRSDDTAVYYCARWREFDFFDYWGQGTTLTVSS

SEQ ID NO: 29 - protein, 118 aa, Artificial Sequence
  humanized VH chain
QVQLVQSGAEVKKPGASVKVSCKASGYTFTSHWIHWVRQAPGQGLEWMGRIEPNSGGTLYAQKFQGRVTMTRDTSISTAYMELSRLRSDDTAVYYCARWREFDFFDYWGQGTTLTVSS

SEQ ID NO: 30 - protein, 118 aa, Artificial Sequence
  humanized VH chain
QVQLVQSGAEVKKPGASVKVSCKASGYTFTSHWIHWVRQAPGQGLEWIGRIEPNSGGTLYNEKFKGRVTMTRDTSTSTVYMELSSLRSEDTAVYYCARWREFDFFDYWGAGTTVTVSS

SEQ ID NO: 31 - protein, 5 aa, Artificial Sequence
  linker
GGGGS

SEQ ID NO: 32 - protein, 15 aa, Artificial Sequence
  linker
GGGGSGGGGSGGGGS

SEQ ID NO: 33 - protein, 25 aa, Artificial Sequence
  GGGGSGGGGS GASAAGGGGS GGGGS
GGGGSGGGGSGASAAGGGGSGGGGS

SEQ ID NO: 34 - protein, 290 aa, Artificial Sequence
  Tagged humanized scFv
MRRMQLLLLIALSLALVTNSEVQLVESGGGLVQPGGSLRLSCAASGFNIKDTYIHWVRQAPGKGLEWVARIYPTNGYTRYADSVKGRFTISADTSKNTAYLQMNSLRAEDTAVYYCSRWGGDGFYAMDVWGQGTLVTVSSGGGGSGGGGSGGGGSDIQMTQSPSSLSASVGDRVTITCRASQDVNTAVAWYQQKPGKAPKLLIYSASFLESGVPSRFSGSRSGTDFTLTISSLQPEDFATYYCQQHYTTPPTFGQGTKVEIKAAAKPLPEVTDEYGPGGGGSHHHHHHHH

SEQ ID NO: 35 - protein, 277 aa, Artificial Sequence
  Tagged humanized scFv
MRRMQLLLLIALSLALVTNSEVQLVESGGGLVQPGGSLRLSCAASGFNIKDTYIHWVRQAPGKGLEWVARIYPTNGYTRYADSVKGRFTISADTSKNTAYLQMNSLRAEDTAVYYCSRWGGDGFYAMDVWGQGTLVTVSSGGGGSGGGGSGGGGSDIQMTQSPSSLSASVGDRVTITCRASQDVNTAVAWYQQKPGKAPKLLIYSASFLESGVPSRFSGSRSGTDFTLTISSLQPEDFATYYCQQHYTTPPTFGQGTKVEIKAAAKPLPEVTDEYGP

SEQ ID NO: 36 - protein, 257 aa, Artificial Sequence
  Tagged humanized scFv
EVQLVESGGGLVQPGGSLRLSCAASGFNIKDTYIHWVRQAPGKGLEWVARIYPTNGYTRYADSVKGRFTISADTSKNTAYLQMNSLRAEDTAVYYCSRWGGDGFYAMDVWGQGTLVTVSSGGGGSGGGGSGGGGSDIQMTQSPSSLSASVGDRVTITCRASQDVNTAVAWYQQKPGKAPKLLIYSASFLESGVPSRFSGSRSGTDFTLTISSLQPEDFATYYCQQHYTTPPTFGQGTKVEIKAAAKPLPEVTDEYGP

SEQ ID NO: 37 - protein, 120 aa, Artificial Sequence
  humanized VH chain
EVQLVESGGGLVQPGGSLRLSCAASGFNIKDTYIHWVRQAPGKGLEWVARIYPTNGYTRYADSVKGRFTISADTSKNTAYLQMNSLRAEDTAVYYCSRWGGDGFYAMDVWGQGTLVTVSS

SEQ ID NO: 38 - protein, 107 aa, Artificial Sequence
  humanized VL chain
DIQMTQSPSSLSASVGDRVTITCRASQDVNTAVAWYQQKPGKAPKLLIYSASFLESGVPSRFSGSRSGTDFTLTISSLQPEDFATYYCQQHYTTPPTFGQGTKVEIK

SEQ ID NO: 39 - protein, 33 aa, Saccharomyces cerevisiae
RMKQLEPKVEELLPKNYHLENEVARLKKLVGER

SEQ ID NO: 40 - protein, 14 aa, Saccharomyces cerevisiae
NYHLENEVARLKKL

SEQ ID NO: 41 - protein, 51 aa, Homo sapiens
MDPDLEIRAAFLRQRNTALRTEVAELEQEVQRLENEVSQYETRYGPLGGGK

SEQ ID NO: 42 - protein, 51 aa, Homo sapiens
MDPDLEIEAAFLERENTALETRVAELRQRVQRLRNRVSQYRTRYGPLGGGK

SEQ ID NO: 43 - protein, 10 aa, Homo sapiens
KPLPEVTDEY

SEQ ID NO: 44 - protein, 20 aa, Homo sapiens
  misc_feature (16)..(16): Xaa can be any naturally occurring amino acid
LEKEALKKIIEDQQEXLNKW

SEQ ID NO: 45 - protein, 20 aa, Homo sapiens
LEKEALKKIIEDQQEALNKW

SEQ ID NO: 46 - protein, 113 aa, Artificial Sequence
  humanized VL chain
  Xaa can be any naturally occurring amino acid (24)..(101)
DIVMTQSPDSLAVSLGERATINCXSSQSLLNSRTXKNYLAWYQQKPGQPPKLLIYWASTRXSGVPDRFSGSGSGTDFTLTISSLQAEDVAVYYCKQSYNLXTFGGGTKVEILK

SEQ ID NO: 47 - protein, 120 aa, Artificial Sequence
  humanized VH chain
QVQLVQSGAEVKKPGASVKVSCKASGYTFTHYYIYWVRQAPGQGLEWMGGVNPSNGGTHFNEKFKSRVTMTRDTSISTAYMELSRLRSDDTAVYYCARSEYDYGLGFAYWGQGTLVTVSS

SEQ ID NO: 48 - protein, 112 aa, Artificial Sequence
  humanized VL chain
DIVMTQSPDSLAVSLGERATINCKSSQSLLNSRTPKNYLAWYQQKPGQPPKLLIYWASTRKSGVPDRFSGSGSGTDFTLTISSLQAEDVAVYYCKQSYNLLTFGGGTKVEIK

SEQ ID NO: 49 - protein, 118 aa, Artificial Sequence
  humanized VH chain
EVQLVESGGGLVQPGGSLRLSCAASGFTFSDFWMNWVRQAPGKGLEWVGQIRNKPNNYETYYSDSLKGRFTISRDDSKSITYLQMNSLRAEDTAVYYCTLGNSWFAYWGQGTLVTVSS

SEQ ID NO: 50 - protein, 112 aa, Artificial Sequence
  humanized VL chain
DIVMTQSPDSLAVSLGERATINCRSSQSLLDSRTKKNYLAWYQQKPGQPPKLLIYWASTRESGVPDRFSGSGSGTDFTLTISSLQAEDVAVYYCKQSYNLPTFGGGTKVEIK

SEQ ID NO: 51 - protein, 115 aa, Mus musculus
DIVLTQTPAIMSASPGEKVTMTCSASSSVSYMHWYQQKSGTSPKRWIYDTSKLASGVPTRFSGSGSGTSYSLTISSMEAEDAATYYCQQWSSNPLTFGAGTKLELKRADAAPTVS

SEQ ID NO: 52 - protein, 117 aa, Mus musculus
EVKLQESGPELVKSGASVKMSCKASGYTFTKYVIHWVKQKPGQGLEWIGYINPYNDVSKYNEKFRGKATLTSDKSSSTAYMELSSLTSEDSAVYFCSRNKDYYPMDYWGQGTSVTVS

SEQ ID NO: 53 - protein, 105 aa, Artificial Sequence
  humanized VL chain
EIVLTQSPATLSLSPGERATLSCSASSSVSYMHWYQQKPGQAPRLLIYDTSKLASGIPARFSGSGSGTDFTLTISSLEPEDFAVYYCQQWSSNPLTFGGGTKVEI

SEQ ID NO: 54 - protein, 117 aa, Artificial Sequence
  humanized VH chain
QVQLVQSGAEVKKPGASVKVSCKASGYTFTKYVIHWVRQAPGQGLEWMGYINPYNDVSKYNEKFRGRVTMTTDTSTSTAYMELRSLRSDDTAVYYCARNKDYYPMDYWGQGTTVTVS

SEQ ID NO: 55 - protein, 108 aa, Artificial Sequence
  humanized VL chain
YELIQPSSASVTVGETVKITCSGDQLPKNFAYWFQQKSDKNILLLIYMDNKRPSGIPERFSGSTSGTTATLTISGAQPEDEAAYYCLSSYGDNNDLVFGSGTQLTVLR

SEQ ID NO: 56 - protein, 121 aa, Artificial Sequence
  humanized VH chain
EVYLVESGGDLVQPGSSLKVSCAASGFTFSDFWMYWVRQAPGKGLEWVGRIKNIPNNYATEYADSVRGRFTISRDDSRNSIYLQMNRLRVDDTAIYYCTRAGRFDHFDYWGQGTMVTVSSA

SEQ ID NO: 57 - protein, 106 aa, Artificial Sequence
  humanized VL chain
SYVLTQPSSVSVAPGQTATISCGGHNIGSKNVHWYQQRPGQSPVLVIYQDNKRPSGIPERFSGSNSGNTATLTISGTQAMDEADYYCQVWDNYSVLFGGGTKLTVL

SEQ ID NO: 58 - protein, 120 aa, Artificial Sequence
  humanized VH chain
QVQLVQSGAEVKKPGESLKVSCKASGYTFTSYYMHWVRQAPGQGLEWMGIINPSGGSTSYAQKFQGRVTMTRDTSTSTVYMELSSLRSEDTAVYYCARGSAYYYDFADYWGQGTLVTVSS

SEQ ID NO: 59 - protein, 335 aa, Artificial Sequence
  Fusion protein Escherichia coli and herpes simplex virus
MSRLDKSKVINSALELLNEVGIEGLTTRKLAQKLGVEQPTLYWHVKNKRALLDALAIEMLDRHHTHFCPLKGESWQDFLRNNAKSFRCALLSHRNGAKVHSDTRPTEKQYETLENQLAFLCQQGFSLENALYALSAVGHFTLGCVLEDQEHQVAKEERETPTTDSMPPLLRQAIELFDHQGAEPAFLFGLELIICGLEKQLKCESGSAYSRARTKNNYGSTIEGLLDLPDDDAPEEAGLAAPRLSFLPAGHTRRLSTAPPTDVSLGDELHLDGEDVAMAHADALDDFDLDMLGDGDSPGPGFTPHDSAPYGALDMADFEFEQMFTDALGIDEYGG

SEQ ID NO: 60 - protein, 248 aa, Artificial Sequence
  Fusion protein Escherichia coli and herpes simplex virus
MSRLDKSKVINGALELLNGVGIEGLTTRKLAQKLGVEQPTLYWHVKNKRALLDALPIEMLDRHHTHFCPLEGESWQDFLRNNAKSFRCALLSHRDGAKVHLGTRPTEKQYETLENQLAFLCQQGFSLENALYALSAVGHFTLGCVLEEQEHQVAKEERETPTTDSMPPLLRQAIELFDRQGAEPAFLFGLELIICGLEKQLKCESGGPADALDDFDLDMLPADALDDFDLDMLPADALDDFDLDMLPG

SEQ ID NO: 61 - protein, 248 aa, Artificial Sequence
  Fusion protein Escherichia coli and herpes simplex virus
MSRLDKSKVINSALELLNGVGIEGLTTRKLAQKLGVEQPTLYWHVKNKRALLDALPIEMLDRHHTHSCPLEGESWQDFLRNNAKSYRCALLSHRDGAKVHLGTRPTEKQYETLENQLAFLCQQGFSLENALYALSAVGHFTLGCVLEEQEHQVAKEERETPTTDSMPPLLKQAIELFDRQGAEPAFLFGLELIICGLEKQLKCESGGPTDALDDFDLDMLPADALDDFDLDMLPADALDDFDLDMLPG

SEQ ID NO: 62 - DNA, 19 bp, Escherichia coli
tccctatcagtgatagaga

SEQ ID NO: 63 - DNA, 16 bp, Artificial Sequence
  spacer
acgatgtcgagtttac

SEQ ID NO: 64 - DNA, 379 bp, Artificial Sequence
  TRE sequence
gagtttactccctatcagtgatagagaacgtatgaagagtttactccctatcagtgatagagaacgtatgcagactttactccctatcagtgatagagaacgtataaggagtttactccctatcagtgatagagaacgtatgaccagtttactccctatcagtgatagagaacgtatctacagtttactccctatcagtgatagagaacgtatatccagtttactccctatcagtgatagagaacgtataagctttaggcgtgtacggtgggcgcctataaaagcagagctcgtttagtgaaccgtcagatcgcctggagcaattccacaacacttttgtcttataccaactttccgtaccacttcctaccctcgtaaa

SEQ ID NO: 65 - DNA, 30 bp, Homo sapiens
ggaggaaaaactgtttcatacagaaggcgt

SEQ ID NO: 66 - DNA, 52 bp, Homo sapiens
cagaattaacagtataaattgcatctcttgttcaagagttccctatcactct

SEQ ID NO: 67 - DNA, 110 bp, Homo sapiens
acattttgacacccccataatatttttccagaattaacagtataaattgcatctcttgttcaagagttccctatcactctctttaatcactactcacagtaacctcaact

SEQ ID NO: 68 - DNA, 232 bp, Artificial sequence
  Fusion of human DNA sequences
ggaggaaaaactgtttcatacagaaggcgtggaggaaaaactgtttcatacagaaggcgtggaggaaaaactgtttcatacagaaggcgtggaggaaaaactgtttcatacagaaggcgtggaggaaaaactgtttcatacagaaggcgtggaggaaaaactgtttcatacagaaggcgtcagaattaacagtataaattgcatctcttgttcaagagttccctatcactct

SEQ ID NO: 69 - DNA, 296 bp, Artificial Sequence
  Fusion of human DNA sequences
aggaggaaaaactgtttcatacagaaggcgtaggaggaaaaactgtttcatacagaaggcgtaggaggaaaaactgtttcatacagaaggcgtaggaggaaaaactgtttcatacagaaggcgtaggaggaaaaactgtttcatacagaaggcgtaggaggaaaaactgtttcatacagaaggcgtacattttgacacccccataatatttttccagaattaacagtataaattgcatctcttgttcaagagttccctatcactctctttaatcactactcacagtaacctcaact

SEQ ID NO: 70 - protein, 627 aa, Artificial Sequence
  humanized homo sapiens/mus musculus chimera
MRRMQLLLLIALSLALVTNSEFQVQLVQSGAEVKKPGASVKVSCKASGYTFTHYYIYWVRQAPGQGLEWMGGVNPSNGGTHFNEKFKSRVTMTRDTSISTAYMELSRLRSDDTAVYYCARSEYDYGLGFAYWGQGTLVTVSSGGGGSGGGGSGGGGSDIVMTQSPDSLAVSLGERATINCKSSQSLLNSRTPKNYLAWYQQKPGQPPKLLIYWASTRKSGVPDRFSGSGSGTDFTLTISSLQAEDVAVYYCKQSYNLLTFGGGTKVEIKAAALEKEALKKIIEDQQEALNKWAAAGPGGGGSKILVKQSPMLVAYDNAVNLSCKYSYNLFSREFRASLHKGLDSAVEVCVVYGNYSQQLQVYSKTGFNCDGKLGNESVTFYLQNLYVNQTDIYFCKIEVMAPPPALDNEKSNGTIIHVKGKHLCPSPLFPGPSKPFWVLVVVGGVLACYSLLVTVAFIIFWVRSKRSRGGHSDYMNMTPRRPGPTRKHYQPYAPPRDFAAYRSGGGGSGGGASGGGGSFSRSADAPAYQQGQNQLYNELNLGRREEYDVLDKRRGRDPEMGGKPRRKNPQEGLYNELQKDKMAEAYSEIGMKGERRRGKGHDGLYQGLSTATKDTYGALHMQALPPR

SEQ ID NO: 71 - protein, 532 aa, Artificial Sequence
  humanized homo sapiens/mus musculus chimera
MRRMQLLLLIALSLALVTNSEFQVQLVQSGAEVKKPGASVKVSCKASGYTFTHYYIYWVRQAPGQGLEWMGGVNPSNGGTHFNEKFKSRVTMTRDTSISTAYMELSRLRSDDTAVYYCARSEYDYGLGFAYWGQGTLVTVSSGGGGSGGGGSGGGGSDIVMTQSPDSLAVSLGERATINCKSSQSLLNSRTPKNYLAWYQQKPGQPPKLLIYWASTRKSGVPDRFSGSGSGTDFTLTISSLQAEDVAVYYCKQSYNLLTFGGGTKVEIKAAALEKEALKKIIEDQQEALNKWAAAGPGGGGSTTTPAPRPPTPAPTIASQPLSLRPEACRPAAGGAVHTRGLDFACDIYIWAPLAGTCGVLLLSLVITLYCGGGGSKRGRKKLLYIFKQPFMRPVQTTQEEDGCSCRFPEEEEGGCELGGGGSFSRSADAPAYKQGQNQLYNELNLGRREEYDVLDKRRGRDPEMGGKPRRKNPQEGLYNELQKDKMAEAYSEIGMKGERRRGKGHDGLYQGLSTATKDTYDALHMQALPPR

SEQ ID NO: 72 - protein, 615 aa, Artificial Sequence
  humanized homo sapiens/mus musculus chimera
MRRMQLLLLIALSLALVTNSEFEVQLVESGGGLVQPGGSLRLSCAASGFTFSDFWMNWVRQAPGKGLEWVGQIRNKPNNYETYYSDSLKGRFTISRDDSKSITYLQMNSLRAEDTAVYYCTLGNSWFAYWGQGTLVTVSSGGGGSGGGGSGGGGSDIVMTQSPDSLAVSLGERATINCRSSQSLLDSRTKKNYLAWYQQKPGQPPKLLIYWASTRESGVPDRFSGSGSGTDFTLTISSLQAEDVAVYYCKQSYNLPTFGGGTKVEIKAAAKPLPEVTDEYAAAGPGGGGSKILVKQSPMLVAYDNAVNLSCKYSYNLFSREFRASLHKGLDSAVEVCVVYGNYSQQLQVYSKTGFNCDGKLGNESVTFYLQNLYVNQTDIYFCKIEVMAPPPALDNEKSNGTIIHVKGKHLCPSPLFPGPSKPFWVLVVVGGVLACYSLLVTVAFIIFWVRSKRSRGGHSDYMNMTPRRPGPTRKHYQPYAPPRDFAAYRSGGGGSGGGASGGGGSFSRSADAPAYQQGQNQLYNELNLGRREEYDVLDKRRGRDPEMGGKPRRKNPQEGLYNELQKDKMAEAYSEIGMKGERRRGKGHDGLYQGLSTATKDTYGALHMQALPPR

SEQ ID NO: 73 - protein, 520 aa, Artificial Sequence
  humanized homo sapiens/mus musculus chimera
MRRMQLLLLIALSLALVTNSEFEVQLVESGGGLVQPGGSLRLSCAASGFTFSDFWMNWVRQAPGKGLEWVGQIRNKPNNYETYYSDSLKGRFTISRDDSKSITYLQMNSLRAEDTAVYYCTLGNSWFAYWGQGTLVTVSSGGGGSGGGGSGGGGSDIVMTQSPDSLAVSLGERATINCRSSQSLLDSRTKKNYLAWYQQKPGQPPKLLIYWASTRESGVPDRFSGSGSGTDFTLTISSLQAEDVAVYYCKQSYNLPTFGGGTKVEIKAAAKPLPEVTDEYAAAGPGGGGSTTTPAPRPPTPAPTIASQPLSLRPEACRPAAGGAVHTRGLDFACDIYIWAPLAGTCGVLLLSLVITLYCGGGGSKRGRKKLLYIFKQPFMRPVQTTQEEDGCSCRFPEEEEGGCELGGGGSFSRSADAPAYKQGQNQLYNELNLGRREEYDVLDKRRGRDPEMGGKPRRKNPQEGLYNELQKDKMAEAYSEIGMKGERRRGKGHDGLYQGLSTATKDTYDALHMQALPPR

SEQ ID NO: 74 - protein, 367 aa, Artificial Sequence
  humanized homo sapiens/mus musculus chimera
MRRMQLLLLIALSLALVTNSEFKPLPEVTDEYAAAGPGGGGSKILVKQSPMLVAYDNAVNLSCKYSYNLFSREFRASLHKGLDSAVEVCVVYGNYSQQLQVYSKTGFNCDGKLGNESVTFYLQNLYVNQTDIYFCKIEVMAPPPALDNEKSNGTIIHVKGKHLCPSPLFPGPSKPFWVLVVVGGVLACYSLLVTVAFIIFWVRSKRSRGGHSDYMNMTPRRPGPTRKHYQPYAPPRDFAAYRSGGGGSGGGASGGGGSFSRSADAPAYQQGQNQLYNELNLGRREEYDVLDKRRGRDPEMGGKPRRKNPQEGLYNELQKDKMAEAYSEIGMKGERRRGKGHDGLYQGLSTATKDTYGALHMQALPPR

SEQ ID NO: 75 - protein, 379 aa, Artificial Sequence
  humanized homo sapiens/mus musculus chimera
MRRMQLLLLIALSLALVTNSEFKPLPEVTDEYAAAGPGGGGSKILVKQSPMLVAYDNAVNLSCKYSYNLFSREFRASLHKGLDSAVEVCVVYGNYSQQLQVYSKTGFNCDGKLGNESVTFYLQNLYVNQTDIYFCKIEVMAPPPALDNEKSNGTIIHVKGKHLCPSPLFPGPSKPFWVLVVVGGVLACYSLLVTVAFIIFWVRSKRSRGGGGSKRGRKKLLYIFKQPFMRPVQTTQEEDGCSCRFPEEEEGGCELGGGGSGGGASGGGGSFSRSADAPAYQQGQNQLYNELNLGRREEYDVLDKRRGRDPEMGGKPRRKNPQEGLYNELQKDKMAEAYSEIGMKGERRRGKGHDGLYQGLSTATKDTYGALHMQALPPR

SEQ ID NO: 76 - protein, 375 aa, Artificial Sequence
  humanized homo sapiens/mus musculus chimera
MRRMQLLLLIALSLALVTNSEFEKEALKKIIEDQQESLNKAAAGPGGGGSKILVKQSPMLVAYDNAVNLSCKYSYNLFSREFRASLHKGLDSAVEVCVVYGNYSQQLQVYSKTGFNCDGKLGNESVTFYLQNLYVNQTDIYFCKIEVMAPPPALDNEKSNGTIIHVKGKHLCPSPLFPGPSKPFWVLVVVGGVLACYSLLVTVAFIIFWVRSKRSRGGHSDYMNMTPRRPGPTRKHYQPYAPPRDFAAYRSGGGGSGGGASGGGGSFSRSADAPAYQQGQNQLYNELNLGRREEYDVLDKRRGRDPEMGGKPRRKNPQEGLYNELQKDKMAEAYSEIGMKGERRRGKGHDGLYQGLSTATKDTYGALHMQALPPR

SEQ ID NO: 77 - protein, 387 aa, Artificial Sequence
  humanized homo sapiens/mus musculus chimera
MRRMQLLLLIALSLALVTNSEFEKEALKKIIEDQQESLNKAAAGPGGGGSKILVKQSPMLVAYDNAVNLSCKYSYNLFSREFRASLHKGLDSAVEVCVVYGNYSQQLQVYSKTGFNCDGKLGNESVTFYLQNLYVNQTDIYFCKIEVMAPPPALDNEKSNGTIIHVKGKHLCPSPLFPGPSKPFWVLVVVGGVLACYSLLVTVAFIIFWVRSKRSRGGGGSKRGRKKLLYIFKQPFMRPVQTTQEEDGCSCRFPEEEEGGCELGGGGSGGGASGGGGSFSRSADAPAYQQGQNQLYNELNLGRREEYDVLDKRRGRDPEMGGKPRRKNPQEGLYNELQKDKMAEAYSEIGMKGERRRGKGHDGLYQGLSTATKDTYGALHMQALPPR

SEQ ID NO: 78 - DNA, 1881 bp, Artificial Sequence
  humanized homo sapiens/mus musculus chimera
atgcgccgcatgcagctgctgcttctgatcgctctgagcctggctcttgtgaccaactctgaattccaggtgcagctggtgcagagcggagccgaggtgaagaagcctggagcctctgtgaaggtgagctgcaaggcttctggctacaccttcacccactactacatctactgggtgagacaggctcccggacagggcctggagtggatgggaggcgtgaaccccagcaacggaggcacccacttcaacgagaagttcaagtctcgcgtgaccatgacccgcgacaccagcatctctaccgcttacatggagctgagccgcctgcgctctgatgataccgctgtgtactactgcgctcgcagcgagtacgattacggactgggcttcgcctactggggccagggaaccctggtgaccgtgagctctggaggcggaggcagcggaggcggcggatctggaggcggaggaagcgatatcgtgatgacccagtctcctgatagcctggctgtgagcctgggcgagagagctaccatcaactgcaagagcagccagagcctgctgaactctcgcacccctaagaactaccttgcttggtaccagcagaagcctggacagccccctaagctgctgatctactgggcttctacccgcaagagcggcgtgcccgacagattctctggcagcggaagcggcaccgatttcaccctgaccatcagcagcctgcaggctgaggacgtggccgtgtactactgcaagcagtcttacaacctgctgaccttcggaggcggaaccaaggtggagatcaaggctgccgctctggagaaggaggccctgaagaagatcatcgaggatcagcaggaggctctgaacaagtgggctgccgctgggcccggaggaggcggcagcaagatcctggtcaaacagtcccctatgctggtcgcttacgacaacgccgttaatctgagttgcaaatatagttacaacctgtttagccgggaatttcgcgcatctctccacaagggactggattctgcggttgaggtttgtgtggtctatggcaattatagccagcaactgcaagtgtacagcaaaacaggctttaactgcgacgggaaactcgggaacgaatcagtgaccttctatctgcagaacctgtacgttaaccaaacagatatttacttctgcaagatagaggtgatggctccaccgccagcactggataacgagaagtccaatggaaccatcattcacgtcaaggggaagcatctgtgtccttccccgttgttccctgggccgagcaaacccttttgggtgcttgtggtagttggcggggtattggcctgctattcccttctcgtaactgtggccttcatcatcttctgggtcagatctaagaggtctaggggcgggcatagcgactacatgaacatgacacccaggcggcctggccccactcgcaaacactaccagccatacgcaccaccaagagactttgccgcatatcggagtggtggcggcgggtcaggaggtggagctagcggtggaggaggttccttctctaggtcagctgatgctcccgcctatcagcaaggtcagaaccagctctacaatgagctgaatctgggacgtcgggaggagtacgacgtgctggataaacgaagaggacgcgatcccgagatgggtgggaagcctaggcgcaagaatccccaggaaggcctctacaatgaactgcagaaagacaagatggccgaagcctacagcgagattggcatgaaaggggagcgacggagaggaaagggacatgacgggttgtatcagggtctttccactgcgacaaaggatacctatggggctctgcacatgcaagcactgccacctaga

SEQ ID NO: 79 - DNA, 1596 bp, Artificial Sequence
  humanized homo sapiens/mus musculus chimera
atgcgccgcatgcagctgctgcttctgatcgctctgagcctggctcttgtgaccaactctgaattccaggtgcagctggtgcagagcggagccgaggtgaagaagcctggagcctctgtgaaggtgagctgcaaggcttctggctacaccttcacccactactacatctactgggtgagacaggctcccggacagggcctggagtggatgggaggcgtgaaccccagcaacggaggcacccacttcaacgagaagttcaagtctcgcgtgaccatgacccgcgacaccagcatctctaccgcttacatggagctgagccgcctgcgctctgatgataccgctgtgtactactgcgctcgcagcgagtacgattacggactgggcttcgcctactggggccagggaaccctggtgaccgtgagctctggaggcggaggcagcggaggcggcggatctggaggcggaggaagcgatatcgtgatgacccagtctcctgatagcctggctgtgagcctgggcgagagagctaccatcaactgcaagagcagccagagcctgctgaactctcgcacccctaagaactaccttgcttggtaccagcagaagcctggacagccccctaagctgctgatctactgggcttctacccgcaagagcggcgtgcccgacagattctctggcagcggaagcggcaccgatttcaccctgaccatcagcagcctgcaggctgaggacgtggccgtgtactactgcaagcagtcttacaacctgctgaccttcggaggcggaaccaaggtggagatcaaggctgccgctctggagaaggaggccctgaagaagatcatcgaggatcagcaggaggctctgaacaagtgggctgccgctgggcccggaggaggcgggtcaaccactacccctgctcccaggcctcctacacccgcgccaacgattgccagtcaacctctgtccctgaggcctgaagcctgcagaccagctgcaggcggtgctgtgcatacacggggcttggactttgcctgcgatatctacatctgggcacctcttgccgggacttgtggcgttctcctgctttctctggtcattaccctgtactgtggaggcggcggtagcaaacgcggacggaagaaactgctgtacatcttcaagcagcccttcatgcgccccgtgcagacaacacaggaagaggacggttgcagctgccgatttcccgaagaggaggagggaggctgtgaattgggcggaggaggctccttctctcgcagtgcagatgccccagcgtacaagcaaggccagaaccagctgtacaacgagctcaatctggggcgtagagaggagtatgacgtgctggacaagaggcgaggaagggaccccgagatgggtggcaaaccgcggcgtaagaatccgcaggaaggcctctacaacgagctgcagaaagacaagatggccgaagcctattccgagatagggatgaaaggggaaagacggcgcggtaaagggcacgatgggctctatcagggtctgagcactgcaaccaaggacacgtatgatgccttgcacatgcaagctcttccaccaaga

SEQ ID NO: 80 - DNA, 1845 bp, Artificial Sequence
  humanized homo sapiens/mus musculus chimera
atgcgccgcatgcagctgctgcttctgatcgctctgagcctggctcttgtgaccaactctgaattcgaggtgcaactggtcgaaagtggcggtggtttagttcagcctggtggaagtctacggcttagctgcgcagcatccggtttcacctttagcgacttttggatgaactgggttcggcaggctccgggcaaaggactggagtgggttgggcaaatccgcaacaaaccgaataactacgaaacttattactcagatagcctgaagggtcgattcaccatcagcagggatgattcaaagtcaatcacttacctacagatgaactcattaagagcggaggatactgcggtgtattactgtacactaggtaactcctggttcgcgtattggggacagggcacccttgtaaccgtctccagcggaggcggaggcagcggaggcggcggatctggaggcggaggaagcgacattgttatgacccagagcccggactctctcgctgttagtcttggtgagcgagcgactattaactgccggagcagtcagagtttgttggactctcggacgaaaaagaactacctggcatggtaccagcagaagccgggccaaccacctaaattactgatatattgggcgtcgactcgtgagtcaggggtaccggacaggttttctggaagcggatcaggaacagacttcactttgacgatctcttcgcttcaagccgaggacgttgcggtttattattgtaagcaaagctataatctgccgacatttggtggcggcaccaaggttgaaattaaggctgccgctaagcctctgcctgaagtgaccgatgagtatgctgccgctgggcccggaggaggcggcagcaagatcctggtcaaacagtcccctatgctggtcgcttacgacaacgccgttaatctgagttgcaaatatagttacaacctgtttagccgggaatttcgcgcatctctccacaagggactggattctgcggttgaggtttgtgtggtctatggcaattatagccagcaactgcaagtgtacagcaaaacaggctttaactgcgacgggaaactcgggaacgaatcagtgaccttctatctgcagaacctgtacgttaaccaaacagatatttacttctgcaagatagaggtgatggctccaccgccagcactggataacgagaagtccaatggaaccatcattcacgtcaaggggaagcatctgtgtccttccccgttgttccctgggccgagcaaacccttttgggtgcttgtggtagttggcggggtattggcctgctattcccttctcgtaactgtggccttcatcatcttctgggtcagatctaagaggtctaggggcgggcatagcgactacatgaacatgacacccaggcggcctggccccactcgcaaacactaccagccatacgcaccaccaagagactttgccgcatatcggagtggtggcggcgggtcaggaggtggagctagcggtggaggaggttccttctctaggtcagctgatgctcccgcctatcagcaaggtcagaaccagctctacaatgagctgaatctgggacgtcgggaggagtacgacgtgctggataaacgaagaggacgcgatcccgagatgggtgggaagcctaggcgcaagaatccccaggaaggcctctacaatgaactgcagaaagacaagatggccgaagcctacagcgagattggcatgaaaggggagcgacggagaggaaagggacatgacgggttgtatcagggtctttccactgcgacaaaggatacctatggggctctgcacatgcaagcactgccacctaga

SEQ ID NO: 81 - DNA, 1563 bp, Artificial Sequence
  humanized homo sapiens/mus musculus chimera
atgcgccgcatgcagctgctgcttctgatcgctctgagcctggctcttgtgaccaactctgaattcgaggtgcaactggtcgaaagtggcggtggtttagttcagcctggtggaagtctacggcttagctgcgcagcatccggtttcacctttagcgacttttggatgaactgggttcggcaggctccgggcaaaggactggagtgggttgggcaaatccgcaacaaaccgaataactacgaaacttattactcagatagcctgaagggtcgattcaccatcagcagggatgattcaaagtcaatcacttacctacagatgaactcattaagagcggaggatactgcggtgtattactgtacactaggtaactcctggttcgcgtattggggacagggcacccttgtaaccgtctccagcggaggcggaggcagcggaggcggcggatctggaggcggaggaagcgacattgttatgacccagagcccggactctctcgctgttagtcttggtgagcgagcgactattaactgccggagcagtcagagtttgttggactctcggacgaaaaagaactacctggcatggtaccagcagaagccgggccaaccacctaaattactgatatattgggcgtcgactcgtgagtcaggggtaccggacaggttttctggaagcggatcaggaacagacttcactttgacgatctcttcgcttcaagccgaggacgttgcggtttattattgtaagcaaagctataatctgccgacatttggtggcggcaccaaggttgaaattaaggctgccgctaagcctctgcctgaagtgaccgatgagtatgctgccgctgggcccggaggaggcggcagcaccactacccctgctcccaggcctcctacacccgcgccaacgattgccagtcaacctctgtccctgaggcctgaagcctgcagaccagctgcaggcggtgctgtgcatacacggggcttggactttgcctgcgatatctacatctgggcacctcttgccgggacttgtggcgttctcctgctttctctggtcattaccctgtactgtggaggcggcggtagcaaacgcggacggaagaaactgctgtacatcttcaagcagcccttcatgcgccccgtgcagacaacacaggaagaggacggttgcagctgccgatttcccgaagaggaggagggaggctgtgaattgggcggaggaggctccttctctcgcagtgcagatgccccagcgtacaagcaaggccagaaccagctgtacaacgagctcaatctggggcgtagagaggagtatgacgtgctggacaagaggcgaggaagggaccccgagatgggtggcaaaccgcggcgtaagaatccgcaggaaggcctctacaacgagctgcagaaagacaagatggccgaagcctattccgagatagggatgaaaggggaaagacggcgcggtaaagggcacgatgggctctatcagggtctgagcactgcaaccaaggacacgtatgatgccttgcacatgcaagctcttccaccaagataa

SEQ ID NO: 82 - DNA, 1101 bp, Artificial Sequence
  humanized homo sapiens/mus musculus chimera
atgcgccgcatgcagctgctgcttctgatcgctctgagcctggctcttgtgaccaactctgaattcaaacccctacctgaagtgactgatgagtatgctgccgctgggcccggaggaggcggcagcaagatcctggtcaaacagtcccctatgctggtcgcttacgacaacgccgttaatctgagttgcaaatatagttacaacctgtttagccgggaatttcgcgcatctctccacaagggactggattctgcggttgaggtttgtgtggtctatggcaattatagccagcaactgcaagtgtacagcaaaacaggctttaactgcgacgggaaactcgggaacgaatcagtgaccttctatctgcagaacctgtacgttaaccaaacagatatttacttctgcaagatagaggtgatggctccaccgccagcactggataacgagaagtccaatggaaccatcattcacgtcaaggggaagcatctgtgtccttccccgttgttccctgggccgagcaaacccttttgggtgcttgtggtagttggcggggtattggcctgctattcccttctcgtaactgtggccttcatcatcttctgggtcagatctaagaggtctaggggcgggcatagcgactacatgaacatgacacccaggcggcctggccccactcgcaaacactaccagccatacgcaccaccaagagactttgccgcatatcggagtggtggcggcgggtcaggaggtggagctagcggtggaggaggttccttctctaggtcagctgatgctcccgcctatcagcaaggtcagaaccagctctacaatgagctgaatctgggacgtcgggaggagtacgacgtgctggataaacgaagaggacgcgatcccgagatgggtgggaagcctaggcgcaagaatccccaggaaggcctctacaatgaactgcagaaagacaagatggccgaagcctacagcgagattggcatgaaaggggagcgacggagaggaaagggacatgacgggttgtatcagggtctttccactgcgacaaaggatacctatggggctctgcacatgcaagcactgccacctaga

SEQ ID NO: 83 - DNA, 1137 bp, Artificial Sequence
  humanized homo sapiens/mus musculus chimera
atgcgccgcatgcagctgctgcttctgatcgctctgagcctggctcttgtgaccaactctgaattcaaacccctacctgaagtgactgatgagtatgctgccgctgggcccggaggaggcggcagcaagatcctggtcaaacagtcccctatgctggtcgcttacgacaacgccgttaatctgagttgcaaatatagttacaacctgtttagccgggaatttcgcgcatctctccacaagggactggattctgcggttgaggtttgtgtggtctatggcaattatagccagcaactgcaagtgtacagcaaaacaggctttaactgcgacgggaaactcgggaacgaatcagtgaccttctatctgcagaacctgtacgttaaccaaacagatatttacttctgcaagatagaggtgatggctccaccgccagcactggataacgagaagtccaatggaaccatcattcacgtcaaggggaagcatctgtgtccttccccgttgttccctgggccgagcaaacccttttgggtgcttgtggtagttggcggggtattggcctgctattcccttctcgtaactgtggccttcatcatcttctgggtcagatctaagaggtctaggggcgggggcgggtcaaaacgcggacggaagaaactgctgtacatcttcaagcagcccttcatgcgccccgtgcagacaacacaggaagaggacggttgcagctgccgatttcccgaagaggaggagggaggctgtgaattgggtggcggcgggtcaggaggtggagctagcggtggaggaggttccttctctaggtcagctgatgctcccgcctatcagcaaggtcagaaccagctctacaatgagctgaatctgggacgtcgggaggagtacgacgtgctggataaacgaagaggacgcgatcccgagatgggtgggaagcctaggcgcaagaatccccaggaaggcctctacaatgaactgcagaaagacaagatggccgaagcctacagcgagattggcatgaaaggggagcgacggagaggaaagggacatgacgggttgtatcagggtctttccactgcgacaaaggatacctatggggctctgcacatgcaagcactgccacctaga

SEQ ID NO: 84 - DNA, 1125 bp, Artificial Sequence
  humanized homo sapiens/mus musculus chimera
atgcgccgcatgcagctgctgcttctgatcgctctgagcctggctcttgtgaccaactctgaattcgagaaagaagcactgaagaaaataatagaagaccaacaagaatccctaaacaaagctgccgctgggcccggaggaggcggcagcaagatcctggtcaaacagtcccctatgctggtcgcttacgacaacgccgttaatctgagttgcaaatatagttacaacctgtttagccgggaatttcgcgcatctctccacaagggactggattctgcggttgaggtttgtgtggtctatggcaattatagccagcaactgcaagtgtacagcaaaacaggctttaactgcgacgggaaactcgggaacgaatcagtgaccttctatctgcagaacctgtacgttaaccaaacagatatttacttctgcaagatagaggtgatggctccaccgccagcactggataacgagaagtccaatggaaccatcattcacgtcaaggggaagcatctgtgtccttccccgttgttccctgggccgagcaaacccttttgggtgcttgtggtagttggcggggtattggcctgctattcccttctcgtaactgtggccttcatcatcttctgggtcagatctaagaggtctaggggcgggcatagcgactacatgaacatgacacccaggcggcctggccccactcgcaaacactaccagccatacgcaccaccaagagactttgccgcatatcggagtggtggcggcgggtcaggaggtggagctagcggtggaggaggttccttctctaggtcagctgatgctcccgcctatcagcaaggtcagaaccagctctacaatgagctgaatctgggacgtcgggaggagtacgacgtgctggataaacgaagaggacgcgatcccgagatgggtgggaagcctaggcgcaagaatccccaggaaggcctctacaatgaactgcagaaagacaagatggccgaagcctacagcgagattggcatgaaaggggagcgacggagaggaaagggacatgacgggttgtatcagggtctttccactgcgacaaaggatacctatggggctctgcacatgcaagcactgccacctaga

SEQ ID NO: 85 - DNA, 1161 bp, Artificial Sequence
  humanized homo sapiens/mus musculus chimera
atgcgccgcatgcagctgctgcttctgatcgctctgagcctggctcttgtgaccaactctgaattcgagaaagaagcactgaagaaaataatagaagaccaacaagaatccctaaacaaagctgccgctgggcccggaggaggcggcagcaagatcctggtcaaacagtcccctatgctggtcgcttacgacaacgccgttaatctgagttgcaaatatagttacaacctgtttagccgggaatttcgcgcatctctccacaagggactggattctgcggttgaggtttgtgtggtctatggcaattatagccagcaactgcaagtgtacagcaaaacaggctttaactgcgacgggaaactcgggaacgaatcagtgaccttctatctgcagaacctgtacgttaaccaaacagatatttacttctgcaagatagaggtgatggctccaccgccagcactggataacgagaagtccaatggaaccatcattcacgtcaaggggaagcatctgtgtccttccccgttgttccctgggccgagcaaacccttttgggtgcttgtggtagttggcggggtattggcctgctattcccttctcgtaactgtggccttcatcatcttctgggtcagatctaagaggtctaggggcgggggcgggtcaaaacgcggacggaagaaactgctgtacatcttcaagcagcccttcatgcgccccgtgcagacaacacaggaagaggacggttgcagctgccgatttcccgaagaggaggagggaggctgtgaattgggtggcggcgggtcaggaggtggagctagcggtggaggaggttccttctctaggtcagctgatgctcccgcctatcagcaaggtcagaaccagctctacaatgagctgaatctgggacgtcgggaggagtacgacgtgctggataaacgaagaggacgcgatcccgagatgggtgggaagcctaggcgcaagaatccccaggaaggcctctacaatgaactgcagaaagacaagatggccgaagcctacagcgagattggcatgaaaggggagcgacggagaggaaagggacatgacgggttgtatcagggtctttccactgcgacaaaggatacctatggggctctgcacatgcaagcactgccacctaga

SEQ ID NO: 86 - protein, 160 aa, Artificial Sequence
  Tagged humanized scFv
MRRMQLLLLIALSLALVTNSGPVPPSTALRELIEELVNITQNQKAPLCNGSMVWSINLTAGMYCAALESLINVSGCSAIEKTQRMLSGFCPHKVSAGQFSSLHVRDTKIEVAQFVKDLLLHLKKLFREGRFNAAAKPLPEVTDEYGPGGGGSHHHHHHHH

SEQ ID NO: 87 - protein, 147 aa, Artificial Sequence
  Tagged humanized scFv
MRRMQLLLLIALSLALVTNSGPVPPSTALRELIEELVNITQNQKAPLCNGSMVWSINLTAGMYCAALESLINVSGCSAIEKTQRMLSGFCPHKVSAGQFSSLHVRDTKIEVAQFVKDLLLHLKKLFREGRFNAAAKPLPEVTDEYGP

SEQ ID NO: 88 - protein, 127 aa, Artificial Sequence
  Tagged humanized scFv
GPVPPSTALRELIEELVNITQNQKAPLCNGSMVWSINLTAGMYCAALESLINVSGCSAIEKTQRMLSGFCPHKVSAGQFSSLHVRDTKIEVAQFVKDLLLHLKKLFREGRFNAAAKPLPEVTDEYGP

SEQ ID NO: 89 - protein, 160 aa, Artificial Sequence
  Tagged humanized scFv
MRRMQLLLLIALSLALVTNSGPVPPSTALRYLIEELVNITQNQKAPLCNYSMVWSINLTAGMYCAALESLINVSGCSAIEKTQRMLSGFCPHKVSAGQFSSLHVRDTKIEVAQFVKDLLLHLKKLFREGRFNAAAKPLPEVTDEYGPGGGGSHHHHHHHH

SEQ ID NO: 90 - protein, 147 aa, Artificial Sequence
  Tagged humanized scFv
MRRMQLLLLIALSLALVTNSGPVPPSTALRYLIEELVNITQNQKAPLCNYSMVWSINLTAGMYCAALESLINVSGCSAIEKTQRMLSGFCPHKVSAGQFSSLHVRDTKIEVAQFVKDLLLHLKKLFREGRFNAAAKPLPEVTDEYGP

SEQ ID NO: 91 - protein, 127 aa, Artificial Sequence
  Tagged humanized scFv
GPVPPSTALRYLIEELVNITQNQKAPLCNYSMVWSINLTAGMYCAALESLINVSGCSAIEKTQRMLSGFCPHKVSAGQFSSLHVRDTKIEVAQFVKDLLLHLKKLFREGRFNAAAKPLPEVTDEYGP

SEQ ID NO: 92 - protein, 160 aa, Artificial Sequence
  Tagged humanized scFv
MRRMQLLLLIALSLALVTNSGPVPPSTALRYLIEELVNITQNQKAPLCNGSAVWSINLTAGMYCAALESLINVSGCSAIEKTQRMLSGFCPHKVSAGQFSSLHVRDTKIEVAQFVKDLLLHLKKLFREGRFNAAAKPLPEVTDEYGPGGGGSHHHHHHHH

SEQ ID NO: 93 - protein, 147 aa, Artificial Sequence
  Tagged humanized scFv
MRRMQLLLLIALSLALVTNSGPVPPSTALRYLIEELVNITQNQKAPLCNGSAVWSINLTAGMYCAALESLINVSGCSAIEKTQRMLSGFCPHKVSAGQFSSLHVRDTKIEVAQFVKDLLLHLKKLFREGRFNAAAKPLPEVTDEYGP

SEQ ID NO: 94 - protein, 127 aa, Artificial Sequence
  Tagged humanized scFv
GPVPPSTALRYLIEELVNITQNQKAPLCNGSAVWSINLTAGMYCAALESLINVSGCSAIEKTQRMLSGFCPHKVSAGQFSSLHVRDTKIEVAQFVKDLLLHLKKLFREGRFNAAAKPLPEVTDEYGP

SEQ ID NO: 95 - protein, 293 aa, Artificial Sequence
  Tagged humanized scFv
MRRMQLLLLIALSLALVTNSEFQVQLQQPGAELVKPGASVKLSCKASGYTFTSHWIHWVKERPGRGLEWIGRIEPNSGGTLYNEKFKTKATLTVDKPSSTAYMQINSLTSEDFAVYYCARWREFDFFDYWGQGTTLTVSSGGGGSGGGGSGGGGSDIVLTQSPATLSVTPGDSVSLSCRASQSISNNLHWYQQKSHESPRLLIKYASQSISGIPSRFSGSGSGTDFTLSISSVETEDFGMYFCQQSNRWPYTFGGGTKLEIKAAAKPLPEVTDEYARGGPGGGGSHHHHHHHH

SEQ ID NO: 96 - protein, 280 aa, Artificial Sequence
  Tagged humanized scFv
MRRMQLLLLIALSLALVTNSEFQVQLQQPGAELVKPGASVKLSCKASGYTFTSHWIHWVKERPGRGLEWIGRIEPNSGGTLYNEKFKTKATLTVDKPSSTAYMQINSLTSEDFAVYYCARWREFDFFDYWGQGTTLTVSSGGGGSGGGGSGGGGSDIVLTQSPATLSVTPGDSVSLSCRASQSISNNLHWYQQKSHESPRLLIKYASQSISGIPSRFSGSGSGTDFTLSISSVETEDFGMYFCQQSNRWPYTFGGGTKLEIKAAAKPLPEVTDEYARGGP

SEQ ID NO: 97 - protein, 260 aa, Artificial Sequence
  Tagged humanized scFv
EFQVQLQQPGAELVKPGASVKLSCKASGYTFTSHWIHWVKERPGRGLEWIGRIEPNSGGTLYNEKFKTKATLTVDKPSSTAYMQINSLTSEDFAVYYCARWREFDFFDYWGQGTTLTVSSGGGGSGGGGSGGGGSDIVLTQSPATLSVTPGDSVSLSCRASQSISNNLHWYQQKSHESPRLLIKYASQSISGIPSRFSGSGSGTDFTLSISSVETEDFGMYFCQQSNRWPYTFGGGTKLEIKAAAKPLPEVTDEYARGGP

SEQ ID NO: 98 - protein, 301 aa, Artificial Sequence
  Tagged humanized scFv
MRRMQLLLLIALSLALVTNSDIVLTQSPAFLSVTPGEKVTLTCQASQSISNNLHWYQQKPDQAPKLLIKYASQSISGVPSRFSGSGSGTDFTLTISSVEAEDFGTYYCQQSNRWPYTFGGGTKLEIKGGGGSGGGGSGASAAGGGGSGGGGSQVQLVQSGAEVVKPGASVKLSCKASGYTFTSHWIHWVKQAPGQGLEWIGRIEPNSGGTLYAQKFQGRATLTVDTSISTAYMEISRLRSDDTAVYYCARWREFDFFDYWGQGTTLTVSSAAAKPLPEVTDEYARGGPGGGGSHHHHHHHH

SEQ ID NO: 99 - protein, 288 aa, Artificial Sequence
  Tagged humanized scFv
MRRMQLLLLIALSLALVTNSDIVLTQSPAFLSVTPGEKVTLTCQASQSISNNLHWYQQKPDQAPKLLIKYASQSISGVPSRFSGSGSGTDFTLTISSVEAEDFGTYYCQQSNRWPYTFGGGTKLEIKGGGGSGGGGSGASAAGGGGSGGGGSQVQLVQSGAEVVKPGASVKLSCKASGYTFTSHWIHWVKQAPGQGLEWIGRIEPNSGGTLYAQKFQGRATLTVDTSISTAYMEISRLRSDDTAVYYCARWREFDFFDYWGQGTTLTVSSAAAKPLPEVTDEYARGGP

SEQ ID NO: 100 - protein, 268 aa, Artificial Sequence
  Tagged humanized scFv
DIVLTQSPAFLSVTPGEKVTLTCQASQSISNNLHWYQQKPDQAPKLLIKYASQSISGVPSRFSGSGSGTDFTLTISSVEAEDFGTYYCQQSNRWPYTFGGGTKLEIKGGGGSGGGGSGASAAGGGGSGGGGSQVQLVQSGAEVVKPGASVKLSCKASGYTFTSHWIHWVKQAPGQGLEWIGRIEPNSGGTLYAQKFQGRATLTVDTSISTAYMEISRLRSDDTAVYYCARWREFDFFDYWGQGTTLTVSSAAAKPLPEVTDEYARGGP

SEQ ID NO: 101 - protein, 301 aa, Artificial Sequence
  Tagged humanized scFv
MRRMQLLLLIALSLALVTNSDIVLTQSPAFLSVTPGEKVTLTCRASQSISNNLHWYQQKPDQAPKLLIKYASQSISGVPSRFSGSGSGTDFTLTISSVEAEDFGTYYCQQSNRWPYTFGGGTKLEIKGGGGSGGGGSGASAAGGGGSGGGGSQVQLVQSGAEVVKPGASVKLSCKASGYTFTSHWIHWVKQAPGQGLEWIGRIEPNSGGTLYNQKFQGRATLTVDKPSSTAYMEISRLRSDDTAVYYCARWREFDFFDYWGQGTTLTVSSAAAKPLPEVTDEYARGGPGGGGSHHHHHHHH

SEQ ID NO: 102 - protein, 288 aa, Artificial Sequence
  Tagged humanized scFv
MRRMQLLLLIALSLALVTNSDIVLTQSPAFLSVTPGEKVTLTCRASQSISNNLHWYQQKPDQAPKLLIKYASQSISGVPSRFSGSGSGTDFTLTISSVEAEDFGTYYCQQSNRWPYTFGGGTKLEIKGGGGSGGGGSGASAAGGGGSGGGGSQVQLVQSGAEVVKPGASVKLSCKASGYTFTSHWIHWVKQAPGQGLEWIGRIEPNSGGTLYNQKFQGRATLTVDKPSSTAYMEISRLRSDDTAVYYCARWREFDFFDYWGQGTTLTVSSAAAKPLPEVTDEYARGGP

SEQ ID NO: 103 - protein, 268 aa, Artificial Sequence
  Tagged humanized scFv
DIVLTQSPAFLSVTPGEKVTLTCRASQSISNNLHWYQQKPDQAPKLLIKYASQSISGVPSRFSGSGSGTDFTLTISSVEAEDFGTYYCQQSNRWPYTFGGGTKLEIKGGGGSGGGGSGASAAGGGGSGGGGSQVQLVQSGAEVVKPGASVKLSCKASGYTFTSHWIHWVKQAPGQGLEWIGRIEPNSGGTLYNQKFQGRATLTVDKPSSTAYMEISRLRSDDTAVYYCARWREFDFFDYWGQGTTLTVSSAAAKPLPEVTDEYARGGP

SEQ ID NO: 104 - protein, 301 aa, Artificial Sequence
  Tagged humanized scFv
MRRMQLLLLIALSLALVTNSDIVLTQSPAFLSVTPGEKVTLTCRASQSISNNLHWYQQKPDQAPKLLIKYASQSISGVPSRFSGSGSGTDFTLTISSVEAEDFGTYYCQQSNRWPYTFGGGTKLEIKGGGGSGGGGSGASAAGGGGSGGGGSQVQLVQSGAEVVKPGASVKLSCKASGYTFTSHWIHWVKQAPGQGLEWIGRIEPNSGGTLYNEKFKTRATLTVDKSISTAYMEISRLRSDDTAVYYCARWREFDFFDYWGQGTTLTVSSAAAKPLPEVTDEYARGGPGGGGSHHHHHHHH

SEQ ID NO: 105 - protein, 288 aa, Artificial Sequence
  Tagged humanized scFv
MRRMQLLLLIALSLALVTNSDIVLTQSPAFLSVTPGEKVTLTCRASQSISNNLHWYQQKPDQAPKLLIKYASQSISGVPSRFSGSGSGTDFTLTISSVEAEDFGTYYCQQSNRWPYTFGGGTKLEIKGGGGSGGGGSGASAAGGGGSGGGGSQVQLVQSGAEVVKPGASVKLSCKASGYTFTSHWIHWVKQAPGQGLEWIGRIEPNSGGTLYNEKFKTRATLTVDKSISTAYMEISRLRSDDTAVYYCARWREFDFFDYWGQGTTLTVSSAAAKPLPEVTDEYARGGP

SEQ ID NO: 106 - protein, 268 aa, Artificial Sequence
  Tagged humanized scFv
DIVLTQSPAFLSVTPGEKVTLTCRASQSISNNLHWYQQKPDQAPKLLIKYASQSISGVPSRFSGSGSGTDFTLTISSVEAEDFGTYYCQQSNRWPYTFGGGTKLEIKGGGGSGGGGSGASAAGGGGSGGGGSQVQLVQSGAEVVKPGASVKLSCKASGYTFTSHWIHWVKQAPGQGLEWIGRIEPNSGGTLYNEKFKTRATLTVDKSISTAYMEISRLRSDDTAVYYCARWREFDFFDYWGQGTTLTVSSAAAKPLPEVTDEYARGGP

SEQ ID NO: 107 - protein, 301 aa, Artificial Sequence
  Tagged humanized scFv
MRRMQLLLLIALSLALVTNSDVVMTQSPAFLSVTPGEKVTITCQASQSISNNLHWYQQKPDQAPKLLIKYASQSISGVPSRFSGSGSGTDFTFTISSLEAEDAATYFCQQSNRWPYTFGGGTKLEIKGGGGSGGGGSGASAAGGGGSGGGGSQVQLVQSGAEVKKPGASVKVSCKASGYTFTSHWIHWVRQAPGQGLEWMGRIEPNSGGTLYAQKFQGRVTMTRDTSISTAYMELSRLRSDDTAVYYCARWREFDFFDYWGQGTTLTVSSAAAKPLPEVTDEYARGGPGGGGSHHHHHHHH

SEQ ID NO: 108 - protein, 288 aa, Artificial Sequence
  Tagged humanized scFv
MRRMQLLLLIALSLALVTNSDVVMTQSPAFLSVTPGEKVTITCQASQSISNNLHWYQQKPDQAPKLLIKYASQSISGVPSRFSGSGSGTDFTFTISSLEAEDAATYFCQQSNRWPYTFGGGTKLEIKGGGGSGGGGSGASAAGGGGSGGGGSQVQLVQSGAEVKKPGASVKVSCKASGYTFTSHWIHWVRQAPGQGLEWMGRIEPNSGGTLYAQKFQGRVTMTRDTSISTAYMELSRLRSDDTAVYYCARWREFDFFDYWGQGTTLTVSSAAAKPLPEVTDEYARGGP

SEQ ID NO: 109 - protein, 268 aa, Artificial Sequence
  Tagged humanized scFv
DVVMTQSPAFLSVTPGEKVTITCQASQSISNNLHWYQQKPDQAPKLLIKYASQSISGVPSRFSGSGSGTDFTFTISSLEAEDAATYFCQQSNRWPYTFGGGTKLEIKGGGGSGGGGSGASAAGGGGSGGGGSQVQLVQSGAEVKKPGASVKVSCKASGYTFTSHWIHWVRQAPGQGLEWMGRIEPNSGGTLYAQKFQGRVTMTRDTSISTAYMELSRLRSDDTAVYYCARWREFDFFDYWGQGTTLTVSSAAAKPLPEVTDEYARGGP

SEQ ID NO: 110 - protein, 302 aa, Artificial Sequence
  Tagged humanized scFv
MRRMQLLLLIALSLALVTNSGQIVLTQSPATLSLSPGERATLSCRASQSISNNLHWYQQKPGQAPRLLIKYASQSISGVPDRFSGSGSGTDFTLTISRLEPEDFAVYYCQQSNRWPYTFGGGTKLEIKGGGGSGGGGSGASAAGGGGSGGGGSQVQLVQSGAEVKKPGASVKVSCKASGYTFTSHWIHWVRQAPGQGLEWIGRIEPNSGGTLYNEKFKGRVTMTRDTSTSTVYMELSSLRSEDTAVYYCARWREFDFFDYWGAGTTVTVSSAAAKPLPEVTDEYARGGPGGGGSHHHHHHHH

SEQ ID NO: 111 - protein, 289 aa, Artificial Sequence
  Tagged humanized scFv
MRRMQLLLLIALSLALVTNSGQIVLTQSPATLSLSPGERATLSCRASQSISNNLHWYQQKPGQAPRLLIKYASQSISGVPDRFSGSGSGTDFTLTISRLEPEDFAVYYCQQSNRWPYTFGGGTKLEIKGGGGSGGGGSGASAAGGGGSGGGGSQVQLVQSGAEVKKPGASVKVSCKASGYTFTSHWIHWVRQAPGQGLEWIGRIEPNSGGTLYNEKFKGRVTMTRDTSTSTVYMELSSLRSEDTAVYYCARWREFDFFDYWGAGTTVTVSSAAAKPLPEVTDEYARGGP

SEQ ID NO: 112 - protein, 269 aa, Artificial Sequence
  Tagged humanized scFv
GQIVLTQSPATLSLSPGERATLSCRASQSISNNLHWYQQKPGQAPRLLIKYASQSISGVPDRFSGSGSGTDFTLTISRLEPEDFAVYYCQQSNRWPYTFGGGTKLEIKGGGGSGGGGSGASAAGGGGSGGGGSQVQLVQSGAEVKKPGASVKVSCKASGYTFTSHWIHWVRQAPGQGLEWIGRIEPNSGGTLYNEKFKGRVTMTRDTSTSTVYMELSSLRSEDTAVYYCARWREFDFFDYWGAGTTVTVSSAAAKPLPEVTDEYARGGP

SEQ ID NO: 113 - protein, 265 aa, Homo sapiens
FLDSPDRPWNPPTFSPALLVVTEGDNATFTCSFSNTSESFVLNWYRMSPSNQTDKLAAFPEDRSQPGQDCRFRVTQLPNGRDFHMSVVRARRNDSGTYLCGAISLAPKAQIKESLRAELRVTERRAEVPTAHPSPSPRPAGQFQTLVVGVVGGLLGSLVLLVWVLAVICSRAARGTIGARRTGQPLKEDPSAVPVFSVDYGELDFQWREKTPEPPVPCVPEQTEYATIVFPSGMGTSSPARRGSADGPRSAQPLRPEDGHCSWPL

SEQ ID NO: 114 - protein, 123 aa, Artificial Sequence
  humanized VH chain
QVQLVQSGAEVKKPGSSVKVSCKTSGDTFSTYAISWVRQAPGQGLEWMGGIIPIFGKAHYAQKFQGRVTITADESTSTAYMELSSLRSEDTAVYFCARKFHFVSGSPFGMDVWGQGTTVTVSS

SEQ ID NO: 115 - protein, 106 aa, Artificial Sequence
  humanized VL chain
EIVLTQSPATLSLSPGERATLSCRASQSVSSYLAWYQQKPGQAPRLLIYDASNRATGIPARFSGSGSGTDFTLTISSLEPEDFAVYYCQQRSNWPTFGQGTKVEIK

SEQ ID NO: 116 - protein, 117 aa, Artificial Sequence
  humanized VH chain
QVQLVQSGAEVKKPGASVKVSCKASGYTFTDYGFSWVRQAPGQGLEWMGWITAYNGNTNYAQKLQGRVTMTTDTSTSTVYMELRSLRSDDTAVYYCARDYFYGMDVWGQGTTVTVSS

SEQ ID NO: 117 - protein, 107 aa, Artificial Sequence
  humanized VL chain
EIVLTQSPATLSLSPGERATLSCRASQSVSSYLVWYQQKPGQAPRLLIYDASNRATGIPARFSGSGSGTDFTLTISSLEPEDFAVYYCQQRSNWPRTFGQGTKVEIK

SEQ ID NO: 118 - protein, 118 aa, Artificial Sequence
  humanized VH chain
QVQLVQSGAEVKKPGASVKVSCKASGYTFTSYDVHWVRQAPGQRLEWMGWLHADTGITKFSQKFQGRVTITRDTSASTAYMELSSLRSEDTAVYYCARERIQLWFDYWGQGTLVTVSS

SEQ ID NO: 119 - protein, 107 aa, Artificial Sequence
  humanized VL chain
DIQMTQSPSSLSASVGDRVTITCRASQGISSWLAWYQQKPEKAPKSLIYAASSLQSGVPSRFSGSGSGTDFTLTISSLQPEDFATYYCQQYNSYPYTFGQGTKLEIK

SEQ ID NO: 120 - protein, 123 aa, Artificial Sequence
  humanized VH chain
QVQLVQSGAEVKEPGSSVKVSCKASGGTFNSYAISWVRQAPGQGLEWMGGIIPLFGIAHYAQKFQGRVTITADESTNTAYMDLSSLRSEDTAVYYCARKYSYVSGSPFGMDVWGQGTTVTVSS

SEQ ID NO: 121 - protein, 106 aa, Artificial Sequence
  humanized VL chain
EIVLTQSPATLSLSPGERATLSCRASQSVSSYLAWYQQKPGQAPRLLIYDASNRATGIPARFSGSGSGTDFTLTISSLEPEDFAVYYCQQRSNWPTFGQGTRLEIK

SEQ ID NO: 122 - protein, 121 aa, Artificial Sequence
  humanized VH chain
QVQLVQSGAEVKKPGSSVKVSCKASGGTFSSYAINWVRQAPGQGLEWMGGIIPIFGSANYAQKFQDRVTITADESTSAAYMELSSLRSEDTAVYYCARDSSGWSRYYMDVWGQGTTVTVSS

SEQ ID NO: 123 - protein, 106 aa, Artificial Sequence
  humanized VL chain
EIVLTQSPGTLSLSPGERATLSCRASQSVSSSYLAWYQQKPGQAPRLLIYGASSRATGIPDRFSGSGSGTDFTLTISRLEPEDFAVYYCQQYGSSPFGGGTKVEIK

SEQ ID NO: 124 - protein, 120 aa, Artificial Sequence
  humanized VH chain
QVQLVQSGAEVKKPGSSVKVSCKVSGGIFSTYAINWVRQAPGQGLEWMGGIIPIFGTANHAQKFQGRVTITADESTSTAYMELSSLRSEDTAVYYCARDQGIAAALFDYWGQGTLVTVSS

SEQ ID NO: 125 - protein, 108 aa, Artificial Sequence
  humanized VL chain
EIVLTQSPGTLSLSPGERATLSCRASQSVSSSYLAWYQQKPGQAPRLLIYGASSRATGIPDRFSGSGSGTDFTLTISRLEPEDFAVYYCQQYGSSPWTFGQGTKVEIK

SEQ ID NO: 126 - protein, 121 aa, Artificial Sequence
  humanized VH chain
EVQLVESGGGLVQPGRSLRLSCAASGITFDDYGMHWVRQAPGKGLEWVSGISWNRGRIEYADSVKGRFTISRDNAKNSLYLQMNSLRAEDTALYYCAKGRFRYFDWFLDYWGQGTLVTVSS

SEQ ID NO: 127 - protein, 107 aa, Artificial Sequence
  humanized VL chain
AIQLTQSPSSLSASVGDRVTITCRASQGISSALAWYQQKPGKAPKLLIYDASSLESGVPSRFSGSGSGTDFTLTISSLQPEDFATYYCQQFNSYPFTFGPGTKVDIK

SEQ ID NO: 128 - protein, 113 aa, Artificial Sequence
  humanized VH chain
EVQLVESGGGLVQPGRSLRLSCAVSGFTFDDYVVHWVRQAPGKGLEWVSGISGNSGNIGYADSVKGRFTISRDNAKNSLYLQMNSLRAEDTALYYCAVPFDYWGQGTLVTVSS

SEQ ID NO: 129 - protein, 107 aa, Artificial Sequence; identical to SEQ ID NO: 119
  humanized VL chain

SEQ ID NO: 130 - protein, 123 aa, Artificial Sequence
  humanized VH chain
QVQLVQSGAEVKKPGSSVKVSCKTSGDTFSSYAISWVRQAPGQGLEWMGGIIPIFGRAHYAQKFQGRVTITADESTSTAYMELSSLRSEDTAVYFCARKFHFVSGSPFGMDVWGQGTTVTVSS

SEQ ID NO: 131 - protein, 106 aa, Artificial Sequence; identical to SEQ ID NO: 115
  humanized VL chain

SEQ ID NO: 132 - protein, 123 aa, Artificial Sequence
  humanized VH chain
QVQLVQSGAEVKKPGSSVKVSCKTSGGTFSSYAISWVRQAPGQGLEWMGGIIPIFGKAHYAQKFQGRVTITADESTTTAYMELSSLRSEDTAVYYCARKYDYVSGSPFGMDVWGQGTTVTVSS

SEQ ID NO: 133 - protein, 106 aa, Artificial Sequence; identical to SEQ ID NO: 115
  humanized VL chain

SEQ ID NO: 134 - protein, 273 aa, Artificial Sequence
  Tagged humanized scFv
QVQLVQSGAEVKKPGSSVKVSCKTSGDTFSTYAISWVRQAPGQGLEWMGGIIPIFGKAHYAQKFQGRVTITADESTSTAYMELSSLRSEDTAVYFCARKFHFVSGSPFGMDVWGQGTTVTVSSGGGGSGGGGSGGGGSEIVLTQSPATLSLSPGERATLSCRASQSVSSYLAWYQQKPGQAPRLLIYDASNRATGIPARFSGSGSGTDFTLTISSLEPEDFAVYYCQQRSNWPTFGQGTKVEIKAAAKPLPEVTDEYARGGPGGGGSHHHHHH

SEQ ID NO: 135 - protein, 273 aa, Artificial Sequence; identical to SEQ ID NO: 134
  Tagged humanized scFv

SEQ ID NO: 136 - protein, 271 aa, Artificial Sequence
  Tagged humanized scFv
GQVQLVQSGAEVKKPGASVKVSCKASGYTFTDYGFSWVRQAPGQGLEWMGWITAYNGNTNYAQKLQGRVTMTTDTSTSTVYMELRSLRSDDTAVYYCARDYFYGMDVWGQGTTVTVSSGGGGSGGGGSGGGGSEIVLTQSPATLSLSPGERATLSCRASQSVSSYLVWYQQKPGQAPRLLIYDASNRATGIPARFSGSGSGTDFTLTISSLEPEDFAVYYCQQRSNWPRTFGQGTKVEIKAAAKPLPEVTDEYARGGPGGGGSHHHHHHHH

SEQ ID NO: 137 - protein, 280 aa, Artificial Sequence
  Tagged humanized scFv
EIVLTQSPATLSLSPGERATLSCRASQSVSSYLVWYQQKPGQAPRLLIYDASNRATGIPARFSGSGSGTDFTLTISSLEPEDFAVYYCQQRSNWPRTFGQGTKVEIKGGGGSGGGGSGASAAGGGGSGGGGSQVQLVQSGAEVKKPGASVKVSCKASGYTFTDYGFSWVRQAPGQGLEWMGWITAYNGNTNYAQKLQGRVTMTTDTSTSTVYMELRSLRSDDTAVYYCARDYFYGMDVWGQGTTVTVSSAAAKPLPEVTDEYARGGPGGGGSHHHHHHHH

SEQ ID NO: 138 - protein, 272 aa, Artificial Sequence
  Tagged humanized scFv
GQVQLVQSGAEVKKPGASVKVSCKASGYTFTSYDVHWVRQAPGQRLEWMGWLHADTGITKFSQKFQGRVTITRDTSASTAYMELSSLRSEDTAVYYCARERIQLWFDYWGQGTLVTVSSGGGGSGGGGSGGGGSDIQMTQSPSSLSASVGDRVTITCRASQGISSWLAWYQQKPEKAPKSLIYAASSLQSGVPSRFSGSGSGTDFTLTISSLQPEDFATYYCQQYNSYPYTFGQGTKLEIKAAAKPLPEVTDEYARGGPGGGGSHHHHHHHH

SEQ ID NO: 139 - protein, 281 aa, Artificial Sequence
  Tagged humanized scFv
DIQMTQSPSSLSASVGDRVTITCRASQGISSWLAWYQQKPEKAPKSLIYAASSLQSGVPSRFSGSGSGTDFTLTISSLQPEDFATYYCQQYNSYPYTFGQGTKLEIKGGGGSGGGGSGASAAGGGGSGGGGSQVQLVQSGAEVKKPGASVKVSCKASGYTFTSYDVHWVRQAPGQRLEWMGWLHADTGITKFSQKFQGRVTITRDTSASTAYMELSSLRSEDTAVYYCARERIQLWFDYWGQGTLVTVSSAAAKPLPEVTDEYARGGPGGGGSHHHHHHHH

SEQ ID NO: 140 - protein, 276 aa, Artificial Sequence
  Tagged humanized scFv
GQVQLVQSGAEVKEPGSSVKVSCKASGGTFNSYAISWVRQAPGQGLEWMGGIIPLFGIAHYAQKFQGRVTITADESTNTAYMDLSSLRSEDTAVYYCARKYSYVSGSPFGMDVWGQGTTVTVSSGGGGSGGGGSGGGGSEIVLTQSPATLSLSPGERATLSCRASQSVSSYLAWYQQKPGQAPRLLIYDASNRATGIPARFSGSGSGTDFTLTISSLEPEDFAVYYCQQRSNWPTFGQGTRLEIKAAAKPLPEVTDEYARGGPGGGGSHHHHHHHH

SEQ ID NO: 141 - protein, 285 aa, Artificial Sequence
  Tagged humanized scFv
EIVLTQSPATLSLSPGERATLSCRASQSVSSYLAWYQQKPGQAPRLLIYDASNRATGIPARFSGSGSGTDFTLTISSLEPEDFAVYYCQQRSNWPTFGQGTRLEIKGGGGSGGGGSGASAAGGGGSGGGGSQVQLVQSGAEVKEPGSSVKVSCKASGGTFNSYAISWVRQAPGQGLEWMGGIIPLFGIAHYAQKFQGRVTITADESTNTAYMDLSSLRSEDTAVYYCARKYSYVSGSPFGMDVWGQGTTVTVSSAAAKPLPEVTDEYARGGPGGGGSHHHHHHHH

SEQ ID NO: 142 - protein, 274 aa, Artificial Sequence
  Tagged humanized scFv
GQVQLVQSGAEVKKPGSSVKVSCKASGGTFSSYAINWVRQAPGQGLEWMGGIIPIFGSANYAQKFQDRVTITADESTSAAYMELSSLRSEDTAVYYCARDSSGWSRYYMDVWGQGTTVTVSSGGGGSGGGGSGGGGSEIVLTQSPGTLSLSPGERATLSCRASQSVSSSYLAWYQQKPGQAPRLLIYGASSRATGIPDRFSGSGSGTDFTLTISRLEPEDFAVYYCQQYGSSPFGGGTKVEIKAAAKPLPEVTDEYARGGPGGGGSHHHHHHHH

SEQ ID NO: 143 - protein, 283 aa, Artificial Sequence
  Tagged humanized scFv
EIVLTQSPGTLSLSPGERATLSCRASQSVSSSYLAWYQQKPGQAPRLLIYGASSRATGIPDRFSGSGSGTDFTLTISRLEPEDFAVYYCQQYGSSPFGGGTKVEIKGGGGSGGGGSGASAAGGGGSGGGGSQVQLVQSGAEVKKPGSSVKVSCKASGGTFSSYAINWVRQAPGQGLEWMGGIIPIFGSANYAQKFQDRVTITADESTSAAYMELSSLRSEDTAVYYCARDSSGWSRYYMDVWGQGTTVTVSSAAAKPLPEVTDEYARGGPGGGGSHHHHHHHH

SEQ ID NO: 144 - protein, 275 aa, Artificial Sequence
  Tagged humanized scFv
GQVQLVQSGAEVKKPGSSVKVSCKVSGGIFSTYAINWVRQAPGQGLEWMGGIIPIFGTANHAQKFQGRVTITADESTSTAYMELSSLRSEDTAVYYCARDQGIAAALFDYWGQGTLVTVSSGGGGSGGGGSGGGGSEIVLTQSPGTLSLSPGERATLSCRASQSVSSSYLAWYQQKPGQAPRLLIYGASSRATGIPDRFSGSGSGTDFTLTISRLEPEDFAVYYCQQYGSSPWTFGQGTKVEIKAAAKPLPEVTDEYARGGPGGGGSHHHHHHHH

SEQ ID NO: 145 - protein, 284 aa, Artificial Sequence
  Tagged humanized scFv
EIVLTQSPGTLSLSPGERATLSCRASQSVSSSYLAWYQQKPGQAPRLLIYGASSRATGIPDRFSGSGSGTDFTLTISRLEPEDFAVYYCQQYGSSPWTFGQGTKVEIKGGGGSGGGGSGASAAGGGGSGGGGSQVQLVQSGAEVKKPGSSVKVSCKVSGGIFSTYAINWVRQAPGQGLEWMGGIIPIFGTANHAQKFQGRVTITADESTSTAYMELSSLRSEDTAVYYCARDQGIAAALFDYWGQGTLVTVSSAAAKPLPEVTDEYARGGPGGGGSHHHHHHHH

SEQ ID NO: 146 - protein, 275 aa, Artificial Sequence
  Tagged humanized scFv
GEVQLVESGGGLVQPGRSLRLSCAASGITFDDYGMHWVRQAPGKGLEWVSGISWNRGRIEYADSVKGRFTISRDNAKNSLYLQMNSLRAEDTALYYCAKGRFRYFDWFLDYWGQGTLVTVSSGGGGSGGGGSGGGGSAIQLTQSPSSLSASVGDRVTITCRASQGISSALAWYQQKPGKAPKLLIYDASSLESGVPSRFSGSGSGTDFTLTISSLQPEDFATYYCQQFNSYPFTFGPGTKVDIKAAAKPLPEVTDEYARGGPGGGGSHHHHHHHH

SEQ ID NO: 147 - protein, 284 aa, Artificial Sequence
  Tagged humanized scFv
AIQLTQSPSSLSASVGDRVTITCRASQGISSALAWYQQKPGKAPKLLIYDASSLESGVPSRFSGSGSGTDFTLTISSLQPEDFATYYCQQFNSYPFTFGPGTKVDIKGGGGSGGGGSGASAAGGGGSGGGGSEVQLVESGGGLVQPGRSLRLSCAASGITFDDYGMHWVRQAPGKGLEWVSGISWNRGRIEYADSVKGRFTISRDNAKNSLYLQMNSLRAEDTALYYCAKGRFRYFDWFLDYWGQGTLVTVSSAAAKPLPEVTDEYARGGPGGGGSHHHHHHHH

SEQ ID NO: 148 - protein, 266 aa, Artificial Sequence
  Tagged humanized scFv
EVQLVESGGGLVQPGRSLRLSCAVSGFTFDDYVVHWVRQAPGKGLEWVSGISGNSGNIGYADSVKGRFTISRDNAKNSLYLQMNSLRAEDTALYYCAVPFDYWGQGTLVTVSSGGGGSGGGGSGGGGSDIQMTQSPSSLSASVGDRVTITCRASQGISSWLAWYQQKPEKAPKSLIYAASSLQSGVPSRFSGSGSGTDFTLTISSLQPEDFATYYCQQYNSYPYTFGQGTKLEIKAAAKPLPEVTDEYARGGPGGGGSHHHHHHHH

SEQ ID NO: 149 - protein, 276 aa, Artificial Sequence
  Tagged humanized scFv
DIQMTQSPSSLSASVGDRVTITCRASQGISSWLAWYQQKPEKAPKSLIYAASSLQSGVPSRFSGSGSGTDFTLTISSLQPEDFATYYCQQYNSYPYTFGQGTKLEIKGGGGSGGGGSGASAAGGGGSGGGGSEVQLVESGGGLVQPGRSLRLSCAVSGFTFDDYVVHWVRQAPGKGLEWVSGISGNSGNIGYADSVKGRFTISRDNAKNSLYLQMNSLRAEDTALYYCAVPFDYWGQGTLVTVSSAAAKPLPEVTDEYARGGPGGGGSHHHHHHHH

SEQ ID NO: 150 - protein, 276 aa, Artificial Sequence
  Tagged humanized scFv
GQVQLVQSGAEVKKPGSSVKVSCKTSGDTFSSYAISWVRQAPGQGLEWMGGIIPIFGRAHYAQKFQGRVTITADESTSTAYMELSSLRSEDTAVYFCARKFHFVSGSPFGMDVWGQGTTVTVSSGGGGSGGGGSGGGGSEIVLTQSPATLSLSPGERATLSCRASQSVSSYLAWYQQKPGQAPRLLIYDASNRATGIPARFSGSGSGTDFTLTISSLEPEDFAVYYCQQRSNWPTFGQGTKVEIKAAAKPLPEVTDEYARGGPGGGGSHHHHHHHH

SEQ ID NO: 151 - protein, 285 aa, Artificial Sequence
  Tagged humanized scFv
EIVLTQSPATLSLSPGERATLSCRASQSVSSYLAWYQQKPGQAPRLLIYDASNRATGIPARFSGSGSGTDFTLTISSLEPEDFAVYYCQQRSNWPTFGQGTKVEIKGGGGSGGGGSGASAAGGGGSGGGGSQVQLVQSGAEVKKPGSSVKVSCKTSGDTFSSYAISWVRQAPGQGLEWMGGIIPIFGRAHYAQKFQGRVTITADESTSTAYMELSSLRSEDTAVYFCARKFHFVSGSPFGMDVWGQGTTVTVSSAAAKPLPEVTDEYARGGPGGGGSHHHHHHHH

SEQ ID NO: 152 - protein, 276 aa, Artificial Sequence
  Tagged humanized scFv
GQVQLVQSGAEVKKPGSSVKVSCKTSGGTFSSYAISWVRQAPGQGLEWMGGIIPIFGKAHYAQKFQGRVTITADESTTTAYMELSSLRSEDTAVYYCARKYDYVSGSPFGMDVWGQGTTVTVSSGGGGSGGGGSGGGGSEIVLTQSPATLSLSPGERATLSCRASQSVSSYLAWYQQKPGQAPRLLIYDASNRATGIPARFSGSGSGTDFTLTISSLEPEDFAVYYCQQRSNWPTFGQGTKVEIKAAAKPLPEVTDEYARGGPGGGGSHHHHHHHH

SEQ ID NO: 153 - protein, 285 aa, Artificial Sequence
  Tagged humanized scFv
EIVLTQSPATLSLSPGERATLSCRASQSVSSYLAWYQQKPGQAPRLLIYDASNRATGIPARFSGSGSGTDFTLTISSLEPEDFAVYYCQQRSNWPTFGQGTKVEIKGGGGSGGGGSGASAAGGGGSGGGGSQVQLVQSGAEVKKPGSSVKVSCKTSGGTFSSYAISWVRQAPGQGLEWMGGIIPIFGKAHYAQKFQGRVTITADESTTTAYMELSSLRSEDTAVYYCARKYDYVSGSPFGMDVWGQGTTVTVSSAAAKPLPEVTDEYARGGPGGGGSHHHHHHHH

SEQ ID NO: 154 - protein, 118 aa, Artificial Sequence [sequence omitted]

SEQ ID NO: 155 - protein, 107 aa, Artificial Sequence [sequence omitted]

SEQ ID NO: 156 - protein, 274 aa, Artificial Sequence
  Tagged humanized scFv
EVQLVESGGGLVQPGGSLRLSCAASGFTFSDSWIHWVRQAPGKGLEWVAWISPYGGSTYYADSVKGRFTISADTSKNTAYLQMNSLRAEDTAVYYCARRHWPGGFDYWGQGTLVTVSSGGGGSGGGGSGGGGSGGGGSDIQMTQSPSSLSASVGDRVTITCRASQDVSTAVAWYQQKPGKAPKLLIYSASFLYSGVPSRFSGSGSGTDFTLTISSLQPEDFATYYCQQYLYHPATFGQGTKVEIKAAAKPLPEVTDEYARGGPGGGGSHHHHHH

SEQ ID NO: 157 - protein, 279 aa, Artificial Sequence
  Tagged humanized scFv
DIQMTQSPSSLSASVGDRVTITCRASQDVSTAVAWYQQKPGKAPKLLIYSASFLYSGVPSRFSGSGSGTDFTLTISSLQPEDFATYYCQQYLYHPATFGQGTKVEIKGGGGSGGGGSGASAAGGGGSGGGGSEVQLVESGGGLVQPGGSLRLSCAASGFTFSDSWIHWVRQAPGKGLEWVAWISPYGGSTYYADSVKGRFTISADTSKNTAYLQMNSLRAEDTAVYYCARRHWPGGFDYWGQGTLVTVSSAAAKPLPEVTDEYARGGPGGGGSHHHHHH

SEQ ID NO: 158 - protein, 121 aa, Artificial Sequence
  humanized VH chain
EVQLVESGGGLVQPGGSLRLSCAASGFTFSRYWMSWVRQAPGKGLEWVANIKQDGSEKYYVDSVKGRFTISRDNAKNSLYLQMNSLRAEDTAVYYCAREGGWFGELAFDYWGQGTLVTVSS

SEQ ID NO: 159 - protein, 108 aa, Artificial Sequence
  humanized VL chain
EIVLTQSPGTLSLSPGERATLSCRASQRVSSSYLAWYQQKPGQAPRLLIYDASSRATGIPDRFSGSGSGTDFTLTISRLEPEDFAVYYCQQYGSLPWTFGQGTKVEIK

SEQ ID NO: 160 - protein, 278 aa, Artificial Sequence
  Tagged humanized scFv
EVQLVESGGGLVQPGGSLRLSCAASGFTFSRYWMSWVRQAPGKGLEWVANIKQDGSEKYYVDSVKGRFTISRDNAKNSLYLQMNSLRAEDTAVYYCAREGGWFGELAFDYWGQGTLVTVSSGGGGSGGGGSGGGGSGGGGSEIVLTQSPGTLSLSPGERATLSCRASQRVSSSYLAWYQQKPGQAPRLLIYDASSRATGIPDRFSGSGSGTDFTLTISRLEPEDFAVYYCQQYGSLPWTFGQGTKVEIKAAAKPLPEVTDEYARGGPGGGGSHHHHHH

SEQ ID NO: 161 - protein, 283 aa, Artificial Sequence
  Tagged humanized scFv
EIVLTQSPGTLSLSPGERATLSCRASQRVSSSYLAWYQQKPGQAPRLLIYDASSRATGIPDRFSGSGSGTDFTLTISRLEPEDFAVYYCQQYGSLPWTFGQGTKVEIKGGGGSGGGGSGASAAGGGGSGGGGSEVQLVESGGGLVQPGGSLRLSCAASGFTFSRYWMSWVRQAPGKGLEWVANIKQDGSEKYYVDSVKGRFTISRDNAKNSLYLQMNSLRAEDTAVYYCAREGGWFGELAFDYWGQGTLVTVSSAAAKPLPEVTDEYARGGPGGGGSHHHHHH

SEQ ID NO: 162 - protein, 450 aa, Artificial Sequence
  humanized VH chain
EVQLLESGGGLVQPGGSLRLSCAASGFTFSSYIMMWVRQAPGKGLEWVSSIYPSGGITFYADTVKGRFTISRDNSKNTLYLQMNSLRAEDTAVYYCARIKLGTVTTVDYWGQGTLVTVSSASTKGPSVFPLAPSSKSTSGGTAALGCLVKDYFPEPVTVSWNSGALTSGVHTFPAVLQSSGLYSLSSVVTVPSSSLGTQTYICNVNHKPSNTKVDKKVEPKSCDKTHTCPPCPAPELLGGPSVFLFPPKPKDTLMISRTPEVTCVVVDVSHEDPEVKFNWYVDGVEVHNAKTKPREEQYNSTYRVVSVLTVLHQDWLNGKEYKCKVSNKALPAPIEKTISKAKGQPREPQVYTLPPSRDELTKNQVSLTCLVKGFYPSDIAVEWESNGQPENNYKTTPPVLDSDGSFFLYSKLTVDKSRWQQGNVFSCSVMHEALHNHYTQKSLSLSPGK

SEQ ID NO: 163 - protein, 216 aa, Artificial Sequence
  humanized VL chain
QSALTQPASVSGSPGQSITISCTGTSSDVGGYNYVSWYQQHPGKAPKLMIYDVSNRPSGVSNRFSGSKSGNTASLTISGLQAEDEADYYCSSYTSSSTRVFGTGTKVTVLGQPKANPTVTLFPPSSEELQANKATLVCLISDFYPGAVTVAWKADGSPVKAGVETTKPSKQSNNKYAASSYLSLTPEQWKSHRSYSCQVTHEGSTVEKTVAPTECS

SEQ ID NO: 164 - protein, 120 aa, Artificial Sequence
  humanized VH chain
EVQLLESGGGLVQPGGSLRLSCAASGFTFSSYIMMWVRQAPGKGLEWVSSIYPSGGITFYADTVKGRFTISRDNSKNTLYLQMNSLRAEDTAVYYCARIKLGTVTTVDYWGQGTLVTVSS

SEQ ID NO: 165 - protein, 110 aa, Artificial Sequence
  humanized VL chain
QSALTQPASVSGSPGQSITISCTGTSSDVGGYNYVSWYQQHPGKAPKLMIYDVSNRPSGVSNRFSGSKSGNTASLTISGLQAEDEADYYCSSYTSSSTRVFGTGTKVTVL

SEQ ID NO: 166 - protein, 276 aa, Artificial Sequence
  Tagged humanized scFv
EVQLLESGGGLVQPGGSLRLSCAASGFTFSSYIMMWVRQAPGKGLEWVSSIYPSGGITFYADTVKGRFTISRDNSKNTLYLQMNSLRAEDTAVYYCARIKLGTVTTVDYWGQGTLVTVSSGGGGSGGGGSGGGGSQSALTQPASVSGSPGQSITISCTGTSSDVGGYNYVSWYQQHPGKAPKLMIYDVSNRPSGVSNRFSGSKSGNTASLTISGLQAEDEADYYCSSYTSSSTRVFGTGTKVTVLAAAKPLPEVTDEYARGGPGGGGSHHHHHHHH

SEQ ID NO: 167 - protein, 287 aa, Artificial Sequence
  Tagged humanized scFv
GQSALTQPASVSGSPGQSITISCTGTSSDVGGYNYVSWYQQHPGKAPKLMIYDVSNRPSGVSNRFSGSKSGNTASLTISGLQAEDEADYYCSSYTSSSTRVFGTGTKVTVLGGGGSGGGGSGASAAGGGGSGGGGSEVQLLESGGGLVQPGGSLRLSCAASGFTFSSYIMMWVRQAPGKGLEWVSSIYPSGGITFYADTVKGRFTISRDNSKNTLYLQMNSLRAEDTAVYYCARIKLGTVTTVDYWGQGTLVTVSSAAAKPLPEVTDEYARGGPGGGGSHHHHHHHH

SEQ ID NO: 168 - protein, 123 aa, Artificial Sequence
  humanized VH chain
EVQLVESGGGLVQPGRSLRLSCAASGFTFDDYAMHWVRQVPGKGLEWVSGISWIRTGIGYADSVKGRFTIFRDNAKNSLYLQMNSLRAEDTALYYCAKDMKGSGTYGGWFDTWGQGTLVTVSS

SEQ ID NO: 169 - protein, 107 aa, Artificial Sequence
  humanized VL chain
DIQMTQSPSSLSASVGDRVTITCRASQSISSYLNWYQQKPGKAPKLLIYVASSLQSGVPSRFSGSGSGTDFTLTISSLQPEDFATYYCQQSYSTPITFGQGTRLEIK

SEQ ID NO: 170 - protein, 118 aa, Artificial Sequence
  humanized VH chain
QVQLQQSGGGLVKPGASLKLSCVTSGFTFRKFGMSWVRQTSDKRLEWVASISTGGYNTYYSDNVKGRFTISRENAKNTLYLQMSSLKSEDTALYYCTRGYSSTSYAMDYWGQGTTVTV

SEQ ID NO: 171 - protein, 108 aa, Artificial Sequence
  humanized VL chain
DIELTQSPASLSVATGEKVTIRCMTSTDIDDDMNWYQQKPGEPPKFLISEGNTLRPGVPSRFSSSGTGTDFVFTIENTLSEDVGDYYCLQSENVPLTEGDGTKLEKAL

SEQ ID NO: 172 - protein, 116 aa, Artificial Sequence
  humanized VH chain
EVQVLESGGGLVQPGGSLRLSCAASGFTFSSYAMSWVFQAPGKGLEWVSAISGSGGSTNYADSVKGRFTISRDNSKNTLYLQMNSLRAEDTAVYYCAGSSGWSEYWGQGTLVTVSS

SEQ ID NO: 173 - protein, 107 aa, Artificial Sequence
  humanized VL chain
DIQMTQSPSSLSASVGDRVTITCRASQGIRNNLAWYQCKPGKAPKRLIYAASNLQSGVPSRFTGSGSGTEFTLIVSSLQPEDFATYYCLQHHSYPLTSGGGTKVEIK

SEQ ID NO: 174 - protein, 117 aa, Artificial Sequence
  humanized VH chain
EVHLQQSGPELEKPGASVKISCKASGYSFTGYNMNVKQSNGKSLEWIGNIDPYYGDTDYDQKFKGTLTADKSSNTVYMQLQSLTSEDSAVYYCARGAHRDYYAMDYWGQGTSVTVSS

SEQ ID NO: 175 - protein, 107 aa, Artificial Sequence
  humanized VL chain
DIQMTQSPASLSASVGETVTITCRTSENIYIYLAWYQQKQGKSPQLLVYNAKTLAEGVPSRFSGSGSGTQFSLKINGLQPEDFGGYYCQQHYGTPYTFGGGTKLEKK

SEQ ID NO: 176 - protein, 272 aa, Homo sapiens
FTVTVPKDLYVVEYGSNMTIECKFPVEKQLDLAALIVYWEMEDKNIIQFVHGEEDLKVQHSSYRQRARLLKDQLSLGNAALQITDVKLQDAGVYRCMISYGGADYKRITVKVNAPYNKINQRILVVDPVTSEHELTCQAEGYPKAEVIWTSSDHQVLSGKTTTTNSKREEKLFNVTSTLRINTTTNEIFYCTFRRLDPEENHTAELVIPELPLAHPPNERTHLVILGAILLCLGVALTFIFRLRKGRMMDVKKCGIQDTNSKKQSDTHLEET